European Patent Specification EP 3 467 125 B1, published August 30, 2023. Title: USING RNA-GUIDED FOKI NUCLEASES (RFNS) TO INCREASE SPECIFICITY FOR RNA-GUIDED GENOME EDITING. Applicant: THE GENERAL HOSPITAL CORPORATION. Application PCT/US2014/028630. The sequence listing filed with the application follows.

SEQUENCE LISTING (466 sequences)

SEQ ID NO: 1 - DNA, 23 bp, Artificial Sequence
  Description of Artificial Sequence: Synthetic binding site oligonucleotide
gggcacgggcagcttgccggtgg

SEQ ID NO: 2 - DNA, 23 bp, Artificial Sequence
  Description of Artificial Sequence: Synthetic binding site oligonucleotide
gatgccgttcttctgcttgtcgg

SEQ ID NO: 3 - DNA, 23 bp, Artificial Sequence
  Description of Artificial Sequence: Synthetic binding site oligonucleotide
ggtggtgcagatgaacttcaggg

SEQ ID NO: 4 - protein, 583 aa, Planomicrobium okeanokoites
MFLSMVSKIRTFGWVQNPGKFENLKRVVQVFDRNSKVHNEVKNIKIPTLVKESKIQKELVAIMNQHDLIYTYKELVGTGTSIRSEAPCDAIIQATIADQGNKKGYIDNWSSDGFLRWAHALGFIEYINKSDSFVITDVGLAYSKSADGSAIEKEILIEAISSYPPAIRILTLLEDGQHLTKFDLGKNLGFSGESGFTSLPEGILLDTLANAMPKDKGEIRNNWEGSSDKYARMIGGWLDKLGLVKQGKKEFIIPTLGKPDNKEFISHAFKITGEGLKVLRRAKGSTKFTRVPKRVYWEMLATNLTDKEYVRTRRALILEILIKAGSLKIEQIQDNLKKLGFDEVIETIENDIKGLINTGIFIEIKGRFYQLKDHILQFVIPNRGVTKQLVKSELEEKKSELRHKLKYVPHEYIELIEIARNSTQDRILEMKVMEFFMKVYGYRGKHLGGSRKPDGAIYTVGSPIDYGVIVDTKAYSGGYNLPIGQADEMQRYVEENQTRNKHINPNEWWKVYPSSVTEFKFLFVSGHFKGNYKAQLTRLNHITNCNGAVLSVEELLIGGEMIKAGTLTLEEVRRKFNNGEINF

SEQ ID NO: 5 - protein, 1368 aa, Streptococcus pyogenes
MDKKYSIGLAIGTNSVGWAVITDEYKVPSKKFKVLGNTDRHSIKKNLIGALLFDSGETAEATRLKRTARRRYTRRKNRICYLQEIFSNEMAKVDDSFFHRLEESFLVEEDKKHERHPIFGNIVDEVAYHEKYPTIYHLRKKLVDSTDKADLRLIYLALAHMIKFRGHFLIEGDLNPDNSDVDKLFIQLVQTYNQLFEENPINASGVDAKAILSARLSKSRRLENLIAQLPGEKKNGLFGNLIALSLGLTPNFKSNFDLAEDAKLQLSKDTYDDDLDNLLAQIGDQYADLFLAAKNLSDAILLSDILRVNTEITKAPLSASMIKRYDEHHQDLTLLKALVRQQLPEKYKEIFFDQSKNGYAGYIDGGASQEEFYKFIKPILEKMDGTEELLVKLNREDLLRKQRTFDNGSIPHQIHLGELHAILRRQEDFYPFLKDNREKIEKILTFRIPYYVGPLARGNSRFAWMTRKSEETITPWNFEEVVDKGASAQSFIERMTNFDKNLPNEKVLPKHSLLYEYFTVYNELTKVKYVTEGMRKPAFLSGEQKKAIVDLLFKTNRKVTVKQLKEDYFKKIECFDSVEISGVEDRFNASLGTYHDLLKIIKDKDFLDNEENEDILEDIVLTLTLFEDREMIEERLKTYAHLFDDKVMKQLKRRRYTGWGRLSRKLINGIRDKQSGKTILDFLKSDGFANRNFMQLIHDDSLTFKEDIQKAQVSGQGDSLHEHIANLAGSPAIKKGILQTVKVVDELVKVMGRHKPENIVIEMARENQTTQKGQKNSRERMKRIEEGIKELGSQILKEHPVENTQLQNEKLYLYYLQNGRDMYVDQELDINRLSDYDVDAIVPQSFLKDDSIDNKVLTRSDKNRGKSDNVPSEEVVKKMKNYWRQLLNAKLITQRKFDNLTKAERGGLSELDKAGFIKRQLVETRQITKHVAQILDSRMNTKYDENDKLIREVKVITLKSKLVSDFRKDFQFYKVREINNYHHAHDAYLNAVVGTALIKKYPKLESEFVYGDYKVYDVRKMIAKSEQEIGKATAKYFFYSNIMNFFKTEITLANGEIRKRPLIETNGETGEIVWDKGRDFATVRKVLSMPQVNIVKKTEVQTGGFSKESILPKRNSDKLIARKKDWDPKKYGGFDSPTVAYSVLVVAKVEKGKSKKLKSVKELLGITIMERSSFEKNPIDFLEAKGYKEVKKDLIIKLPKYSLFELENGRKRMLASAGELQKGNELALPSKYVNFLYLASHYEKLKGSPEDNEQKQLFVEQHKHYLDEIIEQISEFSKRVILADANLDKVLSAYNKHRDKPIREQAENIIHLFTLTNLGAPAAFKYFDTTIDRKRYTSTKEVLDATLIHQSITGLYETRIDLSQLGGD

SEQ ID NO: 6 - RNA, 262 nt, Artificial Sequence
  Description of Artificial Sequence: Synthetic guide RNA polynucleotide
  modified_base (1)..(20): a, c, u, g, unknown or other and this region may encompass 17-20 nucleotides
  modified_base (63)..(262): a, c, u, g, unknown or other and this region may encompass 0-200 nucleotides
nnnnnnnnnnnnnnnnnnnnguuuuagagcuagaaauagcaaguuaaaauaaggcuaguccgnnnnnnnnnnnnnnnnnnnnnnnnnnnnnnnnnnnnnnnnnnnnnnnnnnnnnnnnnnnnnnnnnnnnnnnnnnnnnnnnnnnnnnnnnnnnnnnnnnnnnnnnnnnnnnnnnnnnnnnnnnnnnnnnnnnnnnnnnnnnnnnnnnnnnnnnnnnnnnnnnnnnnnnnnnnnnnnnnnnnnnnnnnnnnnnnnnnnnnnn

SEQ ID NO: 7 - RNA, 275 nt, Artificial Sequence
  Description of Artificial Sequence: Synthetic guide RNA polynucleotide
  modified_base (1)..(20): a, c, u, g, unknown or other and this region may encompass 17-20 nucleotides
  modified_base (76)..(275): a, c, u, g, unknown or other and this region may encompass 0-200 nucleotides
nnnnnnnnnnnnnnnnnnnnguuuuagagcuaugcugaaaagcauagcaaguuaaaauaaggcuaguccguuaucnnnnnnnnnnnnnnnnnnnnnnnnnnnnnnnnnnnnnnnnnnnnnnnnnnnnnnnnnnnnnnnnnnnnnnnnnnnnnnnnnnnnnnnnnnnnnnnnnnnnnnnnnnnnnnnnnnnnnnnnnnnnnnnnnnnnnnnnnnnnnnnnnnnnnnnnnnnnnnnnnnnnnnnnnnnnnnnnnnnnnnnnnnnnnnnnnnnnnnnn

SEQ ID NO: 8 - RNA, 287 nt, Artificial Sequence
  Description of Artificial Sequence: Synthetic guide RNA polynucleotide
  modified_base (1)..(20): a, c, u, g, unknown or other and this region may encompass 17-20 nucleotides
  modified_base (88)..(287): a, c, u, g, unknown or other and this region may encompass 0-200 nucleotides
nnnnnnnnnnnnnnnnnnnnguuuuagagcuaugcuguuuuggaaacaaaacagcauagcaaguuaaaauaaggcuaguccguuaucnnnnnnnnnnnnnnnnnnnnnnnnnnnnnnnnnnnnnnnnnnnnnnnnnnnnnnnnnnnnnnnnnnnnnnnnnnnnnnnnnnnnnnnnnnnnnnnnnnnnnnnnnnnnnnnnnnnnnnnnnnnnnnnnnnnnnnnnnnnnnnnnnnnnnnnnnnnnnnnnnnnnnnnnnnnnnnnnnnnnnnnnnnnnnnnnnnnnnnnn

SEQ ID NO: 9 - RNA, 296 nt, Artificial Sequence
  Description of Artificial Sequence: Synthetic guide RNA polynucleotide
  modified_base (1)..(20): a, c, u, g, unknown or other and this region may encompass 17-20 nucleotides
  modified_base (97)..(296): a, c, u, g, unknown or other and this region may encompass 0-200 nucleotides
nnnnnnnnnnnnnnnnnnnnguuuuagagcuagaaauagcaaguuaaaauaaggcuaguccguuaucaacuugaaaaaguggcaccgagucggugcnnnnnnnnnnnnnnnnnnnnnnnnnnnnnnnnnnnnnnnnnnnnnnnnnnnnnnnnnnnnnnnnnnnnnnnnnnnnnnnnnnnnnnnnnnnnnnnnnnnnnnnnnnnnnnnnnnnnnnnnnnnnnnnnnnnnnnnnnnnnnnnnnnnnnnnnnnnnnnnnnnnnnnnnnnnnnnnnnnnnnnnnnnnnnnnnnnnnnnnn

SEQ ID NO: 10 - RNA, 96 nt, Artificial Sequence
  Description of Artificial Sequence: Synthetic guide RNA oligonucleotide
  modified_base (1)..(20): a, c, u, g, unknown or other and this region may encompass 17-20 nucleotides
nnnnnnnnnnnnnnnnnnnnguuuaagagcuagaaauagcaaguuuaaauaaggcuaguccguuaucaacuugaaaaaguggcaccgagucggugc

SEQ ID NO: 11 - RNA, 106 nt, Artificial Sequence
  Description of Artificial Sequence: Synthetic guide RNA polynucleotide
  modified_base (1)..(20): a, c, u, g, unknown or other and this region may encompass 17-20 nucleotides
nnnnnnnnnnnnnnnnnnnnguuuuagagcuaugcuggaaacagcauagcaaguuuaaauaaggcuaguccguuaucaacuugaaaaaguggcaccgagucggugc

SEQ ID NO: 12 - RNA, 106 nt, Artificial Sequence
  Description of Artificial Sequence: Synthetic guide RNA polynucleotide
  modified_base (1)..(20): a, c, u, g, unknown or other and this region may encompass 17-20 nucleotides
nnnnnnnnnnnnnnnnnnnnguuuaagagcuaugcuggaaacagcauagcaaguuuaaauaaggcuaguccguuaucaacuugaaaaaguggcaccgagucggugc

SEQ ID NO: 13 - RNA, 32 nt, Artificial Sequence
  Description of Artificial Sequence: Synthetic tracrRNA oligonucleotide
  modified_base (1)..(20): a, c, u, g, unknown or other and this region may encompass 17-20 nucleotides
nnnnnnnnnnnnnnnnnnnnguuuuagagcua

SEQ ID NO: 14 - RNA, 42 nt, Artificial Sequence
  Description of Artificial Sequence: Synthetic tracrRNA oligonucleotide
  modified_base (1)..(20): a, c, u, g, unknown or other and this region may encompass 17-20 nucleotides
nnnnnnnnnnnnnnnnnnnnguuuuagagcuaugcuguuuug

SEQ ID NO: 15 - RNA, 36 nt, Artificial Sequence
  Description of Artificial Sequence: Synthetic tracrRNA oligonucleotide
  modified_base (1)..(20): a, c, u, g, unknown or other and this region may encompass 17-20 nucleotides
nnnnnnnnnnnnnnnnnnnnguuuuagagcuaugcu

SEQ ID NO: 16 - RNA, 79 nt, Artificial Sequence
  Description of Artificial Sequence: Synthetic tracrRNA oligonucleotide
ggaaccauucaaaacagcauagcaaguuaaaauaaggcuaguccguuaucaacuugaaaaaguggcaccgagucggugc

SEQ ID NO: 17 - RNA, 60 nt, Artificial Sequence
  Description of Artificial Sequence: Synthetic tracrRNA oligonucleotide
uagcaaguuaaaauaaggcuaguccguuaucaacuugaaaaaguggcaccgagucggugc

SEQ ID NO: 18 - RNA, 64 nt, Artificial Sequence
  Description of Artificial Sequence: Synthetic tracrRNA oligonucleotide
agcauagcaaguuaaaauaaggcuaguccguuaucaacuugaaaaaguggcaccgagucggugc

SEQ ID NO: 19 - DNA, 16 bp, Artificial Sequence
  Description of Artificial Sequence: Synthetic primer
gtaaaacgacggccag

SEQ ID NO: 20 - RNA, 28 nt, Artificial Sequence
  Description of Artificial Sequence: Synthetic Csy4 RNA binding site oligonucleotide
guucacugccguauaggcagcuaagaaa

SEQ ID NO: 21 - RNA, 252 nt, Artificial Sequence
  Description of Artificial Sequence: Synthetic multiplex guide RNA polynucleotide
  modified_base (21)..(40): a, c, u, g, unknown or other
  modified_base (137)..(156): a, c, u, g, unknown or other
guucacugccguauaggcagnnnnnnnnnnnnnnnnnnnnguuuuagagcuagaaauagcaaguuaaaauaaggcuaguccguuaucaacuugaaaaaguggcaccgagucggugcguucacugccguauaggcagnnnnnnnnnnnnnnnnnnnnguuuuagagcuagaaauagcaaguuaaaauaaggcuaguccguuaucaacuugaaaaaguggcaccgagucggugcguucacugccguauaggcag

SEQ ID NO: 22 - protein, 4 aa, Artificial Sequence
  Description of Artificial Sequence: Synthetic linker peptide
GGGS

SEQ ID NO: 23 - protein, 5 aa, Artificial Sequence
  Description of Artificial Sequence: Synthetic linker peptide
GGGGS

SEQ ID NO: 24 - protein, 1602 aa, Artificial Sequence
  Description of Artificial Sequence: Synthetic FokI-dCas9 polypeptide
MQLVKSELEEKKSELRHKLKYVPHEYIELIEIARNSTQDRILEMKVMEFFMKVYGYRGKHLGGSRKPDGAIYTVGSPIDYGVIVDTKAYSGGYNLPIGQADEMQRYVEENQTRNKHINPNEWWKVYPSSVTEFKFLFVSGHFKGNYKAQLTRLNHITNCNGAVLSVEELLIGGEMIKAGTLTLEEVRRKFNNGEINFGGGGSDKKYSIGLAIGTNSVGWAVITDEYKVPSKKFKVLGNTDRHSIKKNLIGALLFDSGETAEATRLKRTARRRYTRRKNRICYLQEIFSNEMAKVDDSFFHRLEESFLVEEDKKHERHPIFGNIVDEVAYHEKYPTIYHLRKKLVDSTDKADLRLIYLALAHMIKFRGHFLIEGDLNPDNSDVDKLFIQLVQTYNQLFEENPINASGVDAKAILSARLSKSRRLENLIAQLPGEKKNGLFGNLIALSLGLTPNFKSNFDLAEDAKLQLSKDTYDDDLDNLLAQIGDQYADLFLAAKNLSDAILLSDILRVNTEITKAPLSASMIKRYDEHHQDLTLLKALVRQQLPEKYKEIFFDQSKNGYAGYIDGGASQEEFYKFIKPILEKMDGTEELLVKLNREDLLRKQRTFDNGSIPHQIHLGELHAILRRQEDFYPFLKDNREKIEKILTFRIPYYVGPLARGNSRFAWMTRKSEETITPWNFEEVVDKGASAQSFIERMTNFDKNLPNEKVLPKHSLLYEYFTVYNELTKVKYVTEGMRKPAFLSGEQKKAIVDLLFKTNRKVTVKQLKEDYFKKIECFDSVEISGVEDRFNASLGTYHDLLKIIKDKDFLDNEENEDILEDIVLTLTLFEDREMIEERLKTYAHLFDDKVMKQLKRRRYTGWGRLSRKLINGIRDKQSGKTILDFLKSDGFANRNFMQLIHDDSLTFKEDIQKAQVSGQGDSLHEHIANLAGSPAIKKGILQTVKVVDELVKVMGRHKPENIVIEMARENQTTQKGQKNSRERMKRIEEGIKELGSQILKEHPVENTQLQNEKLYLYYLQNGRDMYVDQELDINRLSDYDVDAIVPQSFLKDDSIDNKVLTRSDKNRGKSDNVPSEEVVKKMKNYWRQLLNAKLITQRKFDNLTKAERGGLSELDKAGFIKRQLVETRQITKHVAQILDSRMNTKYDENDKLIREVKVITLKSKLVSDFRKDFQFYKVREINNYHHAHDAYLNAVVGTALIKKYPKLESEFVYGDYKVYDVRKMIAKSEQEIGKATAKYFFYSNIMNFFKTEITLANGEIRKRPLIETNGETGEIVWDKGRDFATVRKVLSMPQVNIVKKTEVQTGGFSKESILPKRNSDKLIARKKDWDPKKYGGFDSPTVAYSVLVVAKVEKGKSKKLKSVKELLGITIMERSSFEKNPIDFLEAKGYKEVKKDLIIKLPKYSLFELENGRKRMLASAGELQKGNELALPSKYVNFLYLASHYEKLKGSPEDNEQKQLFVEQHKHYLDEIIEQISEFSKRVILADANLDKVLSAYNKHRDKPIREQAENIIHLFTLTNLGAPAAFKYFDTTIDRKRYTSTKEVLDATLIHQSITGLYETRIDLSQLGGDGSPKKKRKVSSDYKDHDGDYKDHDIDYKDDDDK

SEQ ID NO: 25 - DNA, 4809 bp, Artificial Sequence
  Description of Artificial Sequence: Synthetic FokI-dCas9 polynucleotide
atgcaactagtcaaaagtgaactggaggagaagaaatctgaacttcgtcataaattgaaatatgtgcctcatgaatatattgaattaattgaaattgccagaaattccactcaggatagaattcttgaaatgaaggtaatggaattttttatgaaagtttatggatatagaggtaaacatttgggtggatcaaggaaaccggacggagcaatttatactgtcggatctcctattgattacggtgtgatcgtggatactaaagcttatagcggaggttataatctgccaattggccaagcagatgaaatgcaacgatatgtcgaagaaaatcaaacacgaaacaaacatatcaaccctaatgaatggtggaaagtctatccatcttctgtaacggaatttaagtttttatttgtgagtggtcactttaaaggaaactacaaagctcagcttacacgattaaatcatatcactaattgtaatggagctgttcttagtgtagaagagcttttaattggtggagaaatgattaaagccggcacattaaccttagaggaagtcagacggaaatttaataacggcgagataaactttggtggcggtggatccgataaaaagtattctattggtttagccatcggcactaattccgttggatgggctgtcataaccgatgaatacaaagtaccttcaaagaaatttaaggtgttggggaacacagaccgtcattcgattaaaaagaatcttatcggtgccctcctattcgatagtggcgaaacggcagaggcgactcgcctgaaacgaaccgctcggagaaggtatacacgtcgcaagaaccgaatatgttacttacaagaaatttttagcaatgagatggccaaagttgacgattctttctttcaccgtttggaagagtccttccttgtcgaagaggacaagaaacatgaacggcaccccatctttggaaacatagtagatgaggtggcatatcatgaaaagtacccaacgatttatcacctcagaaaaaagctagttgactcaactgataaagcggacctgaggttaatctacttggctcttgcccatatgataaagttccgtgggcactttctcattgagggtgatctaaatccggacaactcggatgtcgacaaactgttcatccagttagtacaaacctataatcagttgtttgaagagaaccctataaatgcaagtggcgtggatgcgaaggctattcttagcgcccgcctctctaaatcccgacggctagaaaacctgatcgcacaattacccggagagaagaaaaatgggttgttcggtaaccttatagcgctctcactaggcctgacaccaaattttaagtcgaacttcgacttagctgaagatgccaaattgcagcttagtaaggacacgtacgatgacgatctcgacaatctactggcacaaattggagatcagtatgcggacttatttttggctgccaaaaaccttagcgatgcaatcctcctatctgacatactgagagttaatactgagattaccaaggcgccgttatccgcttcaatgatcaaaaggtacgatgaacatcaccaagacttgacacttctcaaggccctagtccgtcagcaactgcctgagaaatataaggaaatattctttgatcagtcgaaaaacgggtacgcaggttatattgacggcggagcgagtcaagaggaattctacaagtttatcaaacccatattagagaagatggatgggacggaagagttgcttgtaaaactcaatcgcgaagatctactgcgaaagcagcggactttcgacaacggtagcattccacatcaaatccacttaggcgaattgcatgctatacttagaaggcaggaggatttttatccgttcctcaaagacaatcgtgaaaagattgagaaaatcctaacctttcgcataccttactatgtgggacccctggcccgagggaactctcggttcgcatggatgacaagaaagtccgaagaaacgattactccatggaattttgaggaagttgtcgataaaggtgcgtcagctcaatcgttcatcgagaggatgaccaactttgacaagaatttaccgaacgaaaaagtattgcctaagcacagtttactttacgagtatttcacagtgtacaatgaactcacgaaagttaagtatgtcactgagggcatgcgtaaacccgcctttctaagcggagaacagaagaaagcaatagtagatctgttattcaagaccaaccgcaaagtgacagttaagcaattgaaagaggactactttaagaaaattgaatgcttcgattctgtcgagatctccggggtagaagatcgatttaatgcgtcacttggtacgtatcatgacctcctaaagataattaaagataaggacttcctggataacgaagagaatgaagatatcttagaagatatagtgttgactcttaccctctttgaagatcgggaaatgattgaggaaagactaaaaacatacgctcacctgttcgacgataaggttatgaaacagttaaagaggcgtcgctatacgggctggggacgattgtcgcggaaacttatcaacgggataagagacaagcaaagtggtaaaactattctcgattttctaaagagcgacggcttcgccaataggaactttatgcagctgatccatgatgactctttaaccttcaaagaggatatacaaaaggcacaggtttccggacaaggggactcattgcacgaacatattgcgaatcttgctggttcgccagccatcaaaaagggcatactccagacagtcaaagtagtggatgagctagttaaggtcatgggacgtcacaaaccggaaaacattgtaatcgagatggcacgcgaaaatcaaacgactcagaaggggcaaaaaaacagtcgagagcggatgaagagaatagaagagggtattaaagaactgggcagccagatcttaaaggagcatcctgtggaaaatacccaattgcagaacgagaaactttacctctattacctacaaaatggaagggacatgtatgttgatcaggaactggacataaaccgtttatctgattacgacgtcgatgccattgtaccccaatcctttttgaaggacgattcaatcgacaataaagtgcttacacgctcggataagaaccgagggaaaagtgacaatgttccaagcgaggaagtcgtaaagaaaatgaagaactattggcggcagctcctaaatgcgaaactgataacgcaaagaaagttcgataacttaactaaagctgagaggggtggcttgtctgaacttgacaaggccggatttattaaacgtcagctcgtggaaacccgccaaatcacaaagcatgttgcacagatactagattcccgaatgaatacgaaatacgacgagaacgataagctgattcgggaagtcaaagtaatcactttaaagtcaaaattggtgtcggacttcagaaaggattttcaattctataaagttagggagataaataactaccaccatgcgcacgacgcttatcttaatgccgtcgtagggaccgcactcattaagaaatacccgaagctagaaagtgagtttgtgtatggtgattacaaagtttatgacgtccgtaagatgatcgcgaaaagcgaacaggagataggcaaggctacagccaaatacttcttttattctaacattatgaatttctttaagacggaaatcactctggcaaacggagagatacgcaaacgacctttaattgaaaccaatggggagacaggtgaaatcgtatgggataagggccgggacttcgcgacggtgagaaaagttttgtccatgccccaagtcaacatagtaaagaaaactgaggtgcagaccggagggttttcaaaggaatcgattcttccaaaaaggaatagtgataagctcatcgctcgtaaaaaggactgggacccgaaaaagtacggtggcttcgatagccctacagttgcctattctgtcctagtagtggcaaaagttgagaagggaaaatccaagaaactgaagtcagtcaaagaattattggggataacgattatggagcgctcgtcttttgaaaagaaccccatcgacttccttgaggcgaaaggttacaaggaagtaaaaaaggatctcataattaaactaccaaagtatagtctgtttgagttagaaaatggccgaaaacggatgttggctagcgccggagagcttcaaaaggggaacgaactcgcactaccgtctaaatacgtgaatttcctgtatttagcgtcccattacgagaagttgaaaggttcacctgaagataacgaacagaagcaactttttgttgagcagcacaaacattatctcgacgaaatcatagagcaaatttcggaattcagtaagagagtcatcctagctgatgccaatctggacaaagtattaagcgcatacaacaagcacagggataaacccatacgtgagcaggcggaaaatattatccatttgtttactcttaccaacctcggcgctccagccgcattcaagtattttgacacaacgatagatcgcaaacgatacacttctaccaaggaggtgctagacgcgacactgattcaccaatccatcacgggattatatgaaactcggatagatttgtcacagcttgggggtgacggatcccccaagaagaagaggaaagtctcgagcgactacaaagaccatgacggtgattataaagatcatgacatcgattacaaggatgacgatgacaagtga

SEQ ID NO: 26 - protein, 1401 aa, Artificial Sequence
  Description of Artificial Sequence: Synthetic Nls-FokI-dCas9-nls polypeptide
MDKKYSIGLAIGTNSVGWAVITDEYKVPSKKFKVLGNTDRHSIKKNLIGALLFDSGETAEATRLKRTARRRYTRRKNRICYLQEIFSNEMAKVDDSFFHRLEESFLVEEDKKHERHPIFGNIVDEVAYHEKYPTIYHLRKKLVDSTDKADLRLIYLALAHMIKFRGHFLIEGDLNPDNSDVDKLFIQLVQTYNQLFEENPINASGVDAKAILSARLSKSRRLENLIAQLPGEKKNGLFGNLIALSLGLTPNFKSNFDLAEDAKLQLSKDTYDDDLDNLLAQIGDQYADLFLAAKNLSDAILLSDILRVNTEITKAPLSASMIKRYDEHHQDLTLLKALVRQQLPEKYKEIFFDQSKNGYAGYIDGGASQEEFYKFIKPILEKMDGTEELLVKLNREDLLRKQRTFDNGSIPHQIHLGELHAILRRQEDFYPFLKDNREKIEKILTFRIPYYVGPLARGNSRFAWMTRKSEETITPWNFEEVVDKGASAQSFIERMTNFDKNLPNEKVLPKHSLLYEYFTVYNELTKVKYVTEGMRKPAFLSGEQKKAIVDLLFKTNRKVTVKQLKEDYFKKIECFDSVEISGVEDRFNASLGTYHDLLKIIKDKDFLDNEENEDILEDIVLTLTLFEDREMIEERLKTYAHLFDDKVMKQLKRRRYTGWGRLSRKLINGIRDKQSGKTILDFLKSDGFANRNFMQLIHDDSLTFKEDIQKAQVSGQGDSLHEHIANLAGSPAIKKGILQTVKVVDELVKVMGRHKPENIVIEMARENQTTQKGQKNSRERMKRIEEGIKELGSQILKEHPVENTQLQNEKLYLYYLQNGRDMYVDQELDINRLSDYDVDAIVPQSFLKDDSIDNKVLTRSDKNRGKSDNVPSEEVVKKMKNYWRQLLNAKLITQRKFDNLTKAERGGLSELDKAGFIKRQLVETRQITKHVAQILDSRMNTKYDENDKLIREVKVITLKSKLVSDFRKDFQFYKVREINNYHHAHDAYLNAVVGTALIKKYPKLESEFVYGDYKVYDVRKMIAKSEQEIGKATAKYFFYSNIMNFFKTEITLANGEIRKRPLIETNGETGEIVWDKGRDFATVRKVLSMPQVNIVKKTEVQTGGFSKESILPKRNSDKLIARKKDWDPKKYGGFDSPTVAYSVLVVAKVEKGKSKKLKSVKELLGITIMERSSFEKNPIDFLEAKGYKEVKKDLIIKLPKYSLFELENGRKRMLASAGELQKGNELALPSKYVNFLYLASHYEKLKGSPEDNEQKQLFVEQHKHYLDEIIEQISEFSKRVILADANLDKVLSAYNKHRDKPIREQAENIIHLFTLTNLGAPAAFKYFDTTIDRKRYTSTKEVLDATLIHQSITGLYETRIDLSQLGGDGSPKKKRKVSSDYKDHDGDYKDHDIDYKDDDDK

SEQ ID NO: 27 - DNA, 4836 bp, Artificial Sequence
  Description of Artificial Sequence: Synthetic Nls-FokI-dCas9-nls polynucleotide
atgcctaagaagaagcggaaggtgagcagccaacttgtgaagtctgaactcgaggagaaaaaatcagagttgagacacaagttgaagtacgtgccacacgaatacatcgagcttatcgagatcgccagaaacagtacccaggataggatccttgagatgaaagtcatggagttctttatgaaggtctacggttatagaggaaagcaccttggcggtagcagaaagcccgatggcgccatctatactgtcggatctcctatcgattatggggtgatcgtggataccaaagcttactcaggcgggtacaacttgcccataggacaagccgacgagatgcagcggtatgtcgaagagaaccagacgcgcaacaagcacatcaaccccaatgaatggtggaaagtgtacccaagtagtgtgactgagttcaagttcctgtttgtctccggccactttaagggcaattataaagctcagctcactagactcaatcacatcacaaactgcaacggagctgtgttgtcagtggaggagctcctgattggaggcgagatgatcaaagccggcacccttacactggaggaggtgcggcggaagttcaacaatggagagatcaacttcggtggcggtggatccgataaaaagtattctattggtttagccatcggcactaattccgttggatgggctgtcataaccgatgaatacaaagtaccttcaaagaaatttaaggtgttggggaacacagaccgtcattcgattaaaaagaatcttatcggtgccctcctattcgatagtggcgaaacggcagaggcgactcgcctgaaacgaaccgctcggagaaggtatacacgtcgcaagaaccgaatatgttacttacaagaaatttttagcaatgagatggccaaagttgacgattctttctttcaccgtttggaagagtccttccttgtcgaagaggacaagaaacatgaacggcaccccatctttggaaacatagtagatgaggtggcatatcatgaaaagtacccaacgatttatcacctcagaaaaaagctagttgactcaactgataaagcggacctgaggttaatctacttggctcttgcccatatgataaagttccgtgggcactttctcattgagggtgatctaaatccggacaactcggatgtcgacaaactgttcatccagttagtacaaacctataatcagttgtttgaagagaaccctataaatgcaagtggcgtggatgcgaaggctattcttagcgcccgcctctctaaatcccgacggctagaaaacctgatcgcacaattacccggagagaagaaaaatgggttgttcggtaaccttatagcgctctcactaggcctgacaccaaattttaagtcgaacttcgacttagctgaagatgccaaattgcagcttagtaaggacacgtacgatgacgatctcgacaatctactggcacaaattggagatcagtatgcggacttatttttggctgccaaaaaccttagcgatgcaatcctcctatctgacatactgagagttaatactgagattaccaaggcgccgttatccgcttcaatgatcaaaaggtacgatgaacatcaccaagacttgacacttctcaaggccctagtccgtcagcaactgcctgagaaatataaggaaatattctttgatcagtcgaaaaacgggtacgcaggttatattgacggcggagcgagtcaagaggaattctacaagtttatcaaacccatattagagaagatggatgggacggaagagttgcttgtaaaactcaatcgcgaagatctactgcgaaagcagcggactttcgacaacggtagcattccacatcaaatccacttaggcgaattgcatgctatacttagaaggcaggaggatttttatccgttcctcaaagacaatcgtgaaaagattgagaaaatcctaacctttcgcataccttactatgtgggacccctggcccgagggaactctcggttcgcatggatgacaagaaagtccgaagaaacgattactccatggaattttgaggaagttgtcgataaaggtgcgtcagctcaatcgttcatcgagaggatgaccaactttgacaagaatttaccgaacgaaaaagtattgcctaagcacagtttactttacgagtatttcacagtgtacaatgaactcacgaaagttaagtatgtcactgagggcatgcgtaaacccgcctttctaagcggagaacagaagaaagcaatagtagatctgttattcaagaccaaccgcaaagtgacagttaagcaattgaaagaggactactttaagaaaattgaatgcttcgattctgtcgagatctccggggtagaagatcgatttaatgcgtcacttggtacgtatcatgacctcctaaagataattaaagataaggacttcctggataacgaagagaatgaagatatcttagaagatatagtgttgactcttaccctctttgaagatcgggaaatgattgaggaaagactaaaaacatacgctcacctgttcgacgataaggttatgaaacagttaaagaggcgtcgctatacgggctggggacgattgtcgcggaaacttatcaacgggataagagacaagcaaagtggtaaaactattctcgattttctaaagagcgacggcttcgccaataggaactttatgcagctgatccatgatgactctttaaccttcaaagaggatatacaaaaggcacaggtttccggacaaggggactcattgcacgaacatattgcgaatcttgctggttcgccagccatcaaaaagggcatactccagacagtcaaagtagtggatgagctagttaaggtcatgggacgtcacaaaccggaaaacattgtaatcgagatggcacgcgaaaatcaaacgactcagaaggggcaaaaaaacagtcgagagcggatgaagagaatagaagagggtattaaagaactgggcagccagatcttaaaggagcatcctgtggaaaatacccaattgcagaacgagaaactttacctctattacctacaaaatggaagggacatgtatgttgatcaggaactggacataaaccgtttatctgattacgacgtcgatgccattgtaccccaatcctttttgaaggacgattcaatcgacaataaagtgcttacacgctcggataagaaccgagggaaaagtgacaatgttccaagcgaggaagtcgtaaagaaaatgaagaactattggcggcagctcctaaatgcgaaactgataacgcaaagaaagttcgataacttaactaaagctgagaggggtggcttgtctgaacttgacaaggccggatttattaaacgtcagctcgtggaaacccgccaaatcacaaagcatgttgcacagatactagattcccgaatgaatacgaaatacgacgagaacgataagctgattcgggaagtcaaagtaatcactttaaagtcaaaattggtgtcggacttcagaaaggattttcaattctataaagttagggagataaataactaccaccatgcgcacgacgcttatcttaatgccgtcgtagggaccgcactcattaagaaatacccgaagctagaaagtgagtttgtgtatggtgattacaaagtttatgacgtccgtaagatgatcgcgaaaagcgaacaggagataggcaaggctacagccaaatacttcttttattctaacattatgaatttctttaagacggaaatcactctggcaaacggagagatacgcaaacgacctttaattgaaaccaatggggagacaggtgaaatcgtatgggataagggccgggacttcgcgacggtgagaaaagttttgtccatgccccaagtcaacatagtaaagaaaactgaggtgcagaccggagggttttcaaaggaatcgattcttccaaaaaggaatagtgataagctcatcgctcgtaaaaaggactgggacccgaaaaagtacggtggcttcgatagccctacagttgcctattctgtcctagtagtggcaaaagttgagaagggaaaatccaagaaactgaagtcagtcaaagaattattggggataacgattatggagcgctcgtcttttgaaaagaaccccatcgacttccttgaggcgaaaggttacaaggaagtaaaaaaggatctcataattaaactaccaaagtatagtctgtttgagttagaaaatggccgaaaacggatgttggctagcgccggagagcttcaaaaggggaacgaactcgcactaccgtctaaatacgtgaatttcctgtatttagcgtcccattacgagaagttgaaaggttcacctgaagataacgaacagaagcaactttttgttgagcagcacaaacattatctcgacgaaatcatagagcaaatttcggaattcagtaagagagtcatcctagctgatgccaatctggacaaagtattaagcgcatacaacaagcacagggataaacccatacgtgagcaggcggaaaatattatccatttgtttactcttaccaacctcggcgctccagccgcattcaagtattttgacacaacgatagatcgcaaacgatacacttctaccaaggaggtgctagacgcgacactgattcaccaatccatcacgggattatatgaaactcggatagatttgtcacagcttgggggtgacggatcccccaagaagaagaggaaagtctcgagcgactacaaagaccatgacggtgattataaagatcatgacatcgattacaaggatgacgatgacaagtga

SEQ ID NO: 28 - DNA, 23 bp, Artificial Sequence
  Description of Artificial Sequence: Synthetic primer
gagctggacggcgacgtaaacgg

SEQ ID NO: 29 - DNA, 23 bp, Artificial Sequence
  Description of Artificial Sequence: Synthetic primer
cgccggacacgctgaacttgtgg

SEQ ID NO: 30 - DNA, 23 bp, Artificial Sequence
  Description of Artificial Sequence: Synthetic primer
ccggcaagctgcccgtgccctgg

SEQ ID NO: 31 - DNA, 23 bp, Artificial Sequence
  Description of Artificial Sequence: Synthetic primer
ggtcagggtggtcacgagggtgg

SEQ ID NO: 32 - DNA, 23 bp, Artificial Sequence
  Description of Artificial Sequence: Synthetic primer
cgaggagctgttcaccggggtgg

SEQ ID NO: 33 - DNA, 23 bp, Artificial Sequence
  Description of Artificial Sequence: Synthetic primer
ccgtccagctcgaccaggatggg

SEQ ID NO: 34 - DNA, 23 bp, Artificial Sequence
  Description of Artificial Sequence: Synthetic primer
cgaggagctgttcaccggggtgg

SEQ ID NO: 35 - DNA, 23 bp, Artificial Sequence
  Description of Artificial Sequence: Synthetic primer
gccgtccagctcgaccaggatgg

SEQ ID NO: 36 - DNA, 23 bp, Artificial Sequence
  Description of Artificial Sequence: Synthetic primer
ccggcaagctgcccgtgccctgg

SEQ ID NO: 37 - DNA, 23 bp, Artificial Sequence
  Description of Artificial Sequence: Synthetic primer
gtaggtcagggtggtcacgaggg

SEQ ID NO: 38 - DNA, 23 bp, Artificial Sequence
  Description of Artificial Sequence: Synthetic primer
gggcgaggagctgttcaccgggg

SEQ ID NO: 39 - DNA, 23 bp, Artificial Sequence
  Description of Artificial Sequence: Synthetic primer
ccgtccagctcgaccaggatggg

SEQ ID NO: 40 - DNA, 23 bp, Artificial Sequence
  Description of Artificial Sequence: Synthetic primer
agggcgaggagctgttcaccggg

SEQ ID NO: 41 - DNA, 23 bp, Artificial Sequence
  Description of Artificial Sequence: Synthetic primer
ccgtccagctcgaccaggatggg

SEQ ID NO: 42 - DNA, 23 bp, Artificial Sequence
  Description of Artificial Sequence: Synthetic primer
aagggcgaggagctgttcaccgg

SEQ ID NO: 43 - DNA, 23 bp, Artificial Sequence
  Description of Artificial Sequence: Synthetic primer
ccgtccagctcgaccaggatggg

SEQ ID NO: 44 - DNA, 23 bp, Artificial Sequence
  Description of Artificial Sequence: Synthetic primer
aagggcgaggagctgttcaccgg

SEQ ID NO: 45 - DNA, 23 bp, Artificial Sequence
  Description of Artificial Sequence: Synthetic primer
gccgtccagctcgaccaggatgg

SEQ ID NO: 46 - DNA, 23 bp, Artificial Sequence
  Description of Artificial Sequence: Synthetic primer
cagcgtgtccggcgagggcgagg

SEQ ID NO: 47 - DNA, 23 bp, Artificial Sequence
  Description of Artificial Sequence: Synthetic primer
cttcagggtcagcttgccgtagg

SEQ ID NO: 48 - DNA, 23 bp, Artificial Sequence
  Description of Artificial Sequence: Synthetic primer
gggcgaggagctgttcaccgggg

SEQ ID NO: 49 - DNA, 23 bp, Artificial Sequence
  Description of Artificial Sequence: Synthetic primer
cgtcgccgtccagctcgaccagg

SEQ ID NO: 50 - DNA, 23 bp, Artificial Sequence
  Description of Artificial Sequence: Synthetic primer
agggcgaggagctgttcaccggg

SEQ ID NO: 51 - DNA, 23 bp, Artificial Sequence
  Description of Artificial Sequence: Synthetic primer
cgtcgccgtccagctcgaccagg

SEQ ID NO: 52 - DNA, 23 bp, Artificial Sequence
  Description of Artificial Sequence: Synthetic primer
aagggcgaggagctgttcaccgg

SEQ ID NO: 53 - DNA, 23 bp, Artificial Sequence
  Description of Artificial Sequence: Synthetic primer
cgtcgccgtccagctcgaccagg

SEQ ID NO: 54 - DNA, 23 bp, Artificial Sequence
  Description of Artificial Sequence: Synthetic primer
ctgaagttcatctgcaccaccgg

SEQ ID NO: 55 - DNA, 23 bp, Artificial Sequence
  Description of Artificial Sequence: Synthetic primer
gtggtcacgagggtgggccaggg

SEQ ID NO: 56 - DNA, 23 bp, Artificial Sequence
  Description of Artificial Sequence: Synthetic primer
aagttcagcgtgtccggcgaggg

SEQ ID NO: 57 - DNA, 23 bp, Artificial Sequence
  Description of Artificial Sequence: Synthetic primer
cttcagggtcagcttgccgtagg

SEQ ID NO: 58 - DNA, 23 bp, Artificial Sequence
  Description of Artificial Sequence: Synthetic primer
caagttcagcgtgtccggcgagg

SEQ ID NO: 59 - DNA, 23 bp, Artificial Sequence
  Description of Artificial Sequence: Synthetic primer
cttcagggtcagcttgccgtagg

SEQ ID NO: 60 - DNA, 23 bp, Artificial Sequence
  Description of Artificial Sequence: Synthetic primer
ggtgcccatcctggtcgagctgg

SEQ ID NO: 61 - DNA, 23 bp, Artificial Sequence
  Description of Artificial Sequence: Synthetic primer
cgccggacacgctgaacttgtgg

SEQ ID NO: 62 - DNA, 23 bp, Artificial Sequence
  Description of Artificial Sequence: Synthetic primer
gagctggacggcgacgtaaacgg

SEQ ID NO: 63 - DNA, 23 bp, Artificial Sequence
  Description of Artificial Sequence: Synthetic primer
ggcatcgccctcgccctcgccgg

SEQ ID NO: 64 - DNA, 23 bp, Artificial Sequence
  Description of Artificial Sequence: Synthetic primer
ggagcgcaccatcttcttcaagg

SEQ ID NO: 65 - DNA, 23 bp, Artificial Sequence
  Description of Artificial Sequence: Synthetic primer
ctcgaacttcacctcggcgcggg

SEQ ID NO: 66 - DNA, 23 bp, Artificial Sequence
  Description of Artificial Sequence: Synthetic primer
ctgaagttcatctgcaccaccgg

SEQ ID NO: 67 - DNA, 23 bp, Artificial Sequence
  Description of Artificial Sequence: Synthetic primer
gtcagggtggtcacgagggtggg

SEQ ID NO: 68 - DNA, 23 bp, Artificial Sequence
  Description of Artificial Sequence: Synthetic primer
ggccacaagttcagcgtgtccgg

SEQ ID NO: 69 - DNA, 23 bp, Artificial Sequence
  Description of Artificial Sequence: Synthetic primer
cttcagggtcagcttgccgtagg

SEQ ID NO: 70 - DNA, 23 bp, Artificial Sequence
  Description of Artificial Sequence: Synthetic primer
ctcgtgaccaccctgacctacgg

SEQ ID NO: 71 - DNA, 23 bp, Artificial Sequence
  Description of Artificial Sequence: Synthetic primer
cgtgctgcttcatgtggtcgggg

SEQ ID NO: 72 - DNA, 23 bp, Artificial Sequence
  Description of Artificial Sequence: Synthetic primer
ccggcaagctgcccgtgccctgg

SEQ ID NO: 73 - DNA, 23 bp, Artificial Sequence
  Description of Artificial Sequence: Synthetic primer
gctgaagcactgcacgccgtagg

SEQ ID NO: 74 - DNA, 23 bp, Artificial Sequence
  Description of Artificial Sequence: Synthetic primer
agcgtgtccggcgagggcgaggg

SEQ ID NO: 75 - DNA, 23 bp, Artificial Sequence
  Description of Artificial Sequence: Synthetic primer
ggtggtgcagatgaacttcaggg

SEQ ID NO: 76 - DNA, 23 bp, Artificial Sequence
  Description of Artificial Sequence: Synthetic primer
cagcgtgtccggcgagggcgagg

SEQ ID NO: 77 - DNA, 23 bp, Artificial Sequence
  Description of Artificial Sequence: Synthetic primer
ggtggtgcagatgaacttcaggg

SEQ ID NO: 78 - DNA, 23 bp, Artificial Sequence
  Description of Artificial Sequence: Synthetic primer
caccggggtggtgcccatcctgg

SEQ ID NO: 79 - DNA, 23 bp, Artificial Sequence
  Description of Artificial Sequence: Synthetic primer
cgccggacacgctgaacttgtgg

SEQ ID NO: 80 - DNA, 23 bp, Artificial Sequence
  Description of Artificial Sequence: Synthetic primer
ggcgagggcgatgccacctacgg

SEQ ID NO: 81 - DNA, 23 bp, Artificial Sequence
  Description of Artificial Sequence: Synthetic primer
gggcacgggcagcttgccggtgg

SEQ ID NO: 82 - DNA, 23 bp, Artificial Sequence
  Description of Artificial Sequence: Synthetic primer
ctcgtgaccaccctgacctacgg

SEQ ID NO: 83 - DNA, 23 bp, Artificial Sequence
  Description of Artificial Sequence: Synthetic primer
agaagtcgtgctgcttcatgtgg

SEQ ID NO: 84 - DNA, 23 bp, Artificial Sequence
  Description of Artificial Sequence: Synthetic primer
caactacaagacccgcgccgagg

SEQ ID NO: 85 - DNA, 23 bp, Artificial Sequence
  Description of Artificial Sequence: Synthetic primer
cgatgcccttcagctcgatgcgg

SEQ ID NO: 86 - DNA, 23 bp, Artificial Sequence
  Description of Artificial Sequence: Synthetic primer
cccatcctggtcgagctggacgg

SEQ ID NO: 87 - DNA, 23 bp, Artificial Sequence
  Description of Artificial Sequence: Synthetic primer
ggcatcgccctcgccctcgccgg

SEQ ID NO: 88 - DNA, 23 bp, Artificial Sequence
  Description of Artificial Sequence: Synthetic primer
caagttcagcgtgtccggcgagg

SEQ ID NO: 89 - DNA, 23 bp, Artificial Sequence
  Description of Artificial Sequence: Synthetic primer
ggtggtgcagatgaacttcaggg

SEQ ID NO: 90 - DNA, 23 bp, Artificial Sequence
  Description of Artificial Sequence: Synthetic primer
gagctggacggcgacgtaaacgg

SEQ ID NO: 91 - DNA, 23 bp, Artificial Sequence
  Description of Artificial Sequence: Synthetic primer
gaccaggatgggcaccaccccgg

SEQ ID NO: 92 - DNA, 23 bp, Artificial Sequence
  Description of Artificial Sequence: Synthetic primer
accatcttcttcaaggacgacgg

SEQ ID NO: 93 - DNA, 23 bp, Artificial Sequence
  Description of Artificial Sequence: Synthetic primer
cgctcctggacgtagccttcggg

SEQ ID NO: 94 - DNA, 23 bp, Artificial Sequence
  Description of Artificial Sequence: Synthetic primer
ggcgagggcgatgccacctacgg

SEQ ID NO: 95 - DNA, 23 bp, Artificial Sequence
  Description of Artificial Sequence: Synthetic primer
cgccggacacgctgaacttgtgg

SEQ ID NO: 96 - DNA, 23 bp, Artificial Sequence
  Description of Artificial Sequence: Synthetic primer
ttcaagtccgccatgcccgaagg

SEQ ID NO: 97 - DNA, 23 bp, Artificial Sequence
  Description of Artificial Sequence: Synthetic primer
gtcgtgctgcttcatgtggtcgg

SEQ ID NO: 98 - DNA, 23 bp, Artificial Sequence
  Description of Artificial Sequence: Synthetic primer
ttcaagtccgccatgcccgaagg

SEQ ID NO: 99 - DNA, 23 bp, Artificial Sequence
  Description of Artificial Sequence: Synthetic primer
tcgtgctgcttcatgtggtcggg

SEQ ID NO: 100 - DNA, 23 bp, Artificial Sequence
  Description of Artificial Sequence: Synthetic primer
ggccacaagttcagcgtgtccgg

SEQ ID NO: 101 - DNA, 23 bp, Artificial Sequence
  Description of Artificial Sequence: Synthetic primer
cgtcgccgtccagctcgaccagg

SEQ ID NO: 102 - DNA, 23 bp, Artificial Sequence
  Description of Artificial Sequence: Synthetic primer
ctcgtgaccaccctgacctacgg

SEQ ID NO: 103 - DNA, 23 bp, Artificial Sequence
  Description of Artificial Sequence: Synthetic primer
ccagggcacgggcagcttgccgg

SEQ ID NO: 104 - DNA, 23 bp, Artificial Sequence
  Description of Artificial Sequence: Synthetic primer
cagccacaacgtctatatcatgg

SEQ ID NO: 105 - DNA, 23 bp, Artificial Sequence
  Description of Artificial Sequence: Synthetic primer
tgtactccagcttgtgccccagg

SEQ ID NO: 106 - DNA, 23 bp, Artificial Sequence
  Description of Artificial Sequence: Synthetic primer
ggccacaagttcagcgtgtccgg

SEQ ID NO: 107 - DNA, 23 bp, Artificial Sequence
  Description of Artificial Sequence: Synthetic primer
gccgtccagctcgaccaggatgg

SEQ ID NO: 108 - DNA, 23 bp, Artificial Sequence
  Description of Artificial Sequence: Synthetic primer
ggccacaagttcagcgtgtccgg

SEQ ID NO: 109 - DNA, 23 bp, Artificial Sequence
  Description of Artificial Sequence: Synthetic primer
ccgtccagctcgaccaggatggg

SEQ ID NO: 110 - DNA, 23 bp, Artificial Sequence
  Description of Artificial Sequence: Synthetic primer
aagttcagcgtgtccggcgaggg

SEQ ID NO: 111 - DNA, 23 bp, Artificial Sequence
  Description of Artificial Sequence: Synthetic primer
cgtcgccgtccagctcgaccagg

SEQ ID NO: 112 - DNA, 23 bp, Artificial Sequence
  Description of Artificial Sequence: Synthetic primer
cgcgccgaggtgaagttcgaggg

SEQ ID NO: 113 - DNA, 23 bp, Artificial Sequence
  Description of Artificial Sequence: Synthetic primer
gccgtcgtccttgaagaagatgg

SEQ ID NO: 114 - DNA, 23 bp, Artificial Sequence
  Description of Artificial Sequence: Synthetic primer
ccggcaagctgcccgtgccctgg

SEQ ID NO: 115 - DNA, 23 bp, Artificial Sequence
  Description of Artificial Sequence: Synthetic primer
cttcagggtcagcttgccgtagg

SEQ ID NO: 116 - DNA, 23 bp, Artificial Sequence
  Description of Artificial Sequence: Synthetic primer
caagttcagcgtgtccggcgagg

SEQ ID NO: 117 - DNA, 23 bp, Artificial Sequence
  Description of Artificial Sequence: Synthetic primer
gccgtccagctcgaccaggatgg

SEQ ID NO: 118 - DNA, 23 bp, Artificial Sequence
  Description of Artificial Sequence: Synthetic primer
caagttcagcgtgtccggcgagg

SEQ ID NO: 119 - DNA, 23 bp, Artificial Sequence
  Description of Artificial Sequence: Synthetic primer
ccgtccagctcgaccaggatggg

SEQ ID NO: 120 - DNA, 23 bp, Artificial Sequence
  Description of Artificial Sequence: Synthetic primer
aagttcagcgtgtccggcgaggg

SEQ ID NO: 121 - DNA, 23 bp, Artificial Sequence
  Description of Artificial Sequence: Synthetic primer
ccgtccagctcgaccaggatggg

SEQ ID NO: 122 - DNA, 23 bp, Artificial Sequence
  Description of Artificial Sequence: Synthetic primer
agcgtgtccggcgagggcgaggg

SEQ ID NO: 123 - DNA, 23 bp, Artificial Sequence
  Description of Artificial Sequence: Synthetic primer
cgtcgccgtccagctcgaccagg

SEQ ID NO: 124 - DNA, 23 bp, Artificial Sequence
  Description of Artificial Sequence: Synthetic primer
ctgaagttcatctgcaccaccgg

SEQ ID NO: 125 - DNA, 23 bp, Artificial Sequence
  Description of Artificial Sequence: Synthetic primer
ggcatcgccctcgccctcgccgg

SEQ ID NO: 126 - DNA, 23 bp, Artificial Sequence
  Description of Artificial Sequence: Synthetic primer
cagcgtgtccggcgagggcgagg

SEQ ID NO: 127 - DNA, 23 bp, Artificial Sequence
  Description of Artificial Sequence: Synthetic primer
gccgtccagctcgaccaggatgg

SEQ ID NO: 128 - DNA, 23 bp, Artificial Sequence
  Description of Artificial Sequence: Synthetic primer
ggccacaagttcagcgtgtccgg

SEQ ID NO: 129 - DNA, 23 bp, Artificial Sequence
  Description of Artificial Sequence: Synthetic primer
gaccaggatgggcaccaccccgg

SEQ ID NO: 130 - DNA, 23 bp, Artificial Sequence
  Description of Artificial Sequence: Synthetic primer
agcgtgtccggcgagggcgaggg

SEQ ID NO: 131 - DNA, 23 bp, Artificial Sequence
  Description of Artificial Sequence: Synthetic primer
ccgtccagctcgaccaggatggg

SEQ ID NO: 132 - DNA, 23 bp, Artificial Sequence
  Description of Artificial Sequence: Synthetic primer
caactacaagacccgcgccgagg

SEQ ID NO: 133 - DNA, 23 bp, Artificial Sequence
  Description of Artificial Sequence: Synthetic primer
gcgctcctggacgtagccttcgg

SEQ ID NO: 134 - DNA, 23 bp, Artificial Sequence
  Description of Artificial Sequence: Synthetic primer
caactacaagacccgcgccgagg

SEQ ID NO: 135 - DNA, 23 bp, Artificial Sequence
  Description of Artificial Sequence: Synthetic primer
cgctcctggacgtagccttcggg

SEQ ID NO: 136 - DNA, 23 bp, Artificial Sequence
  Description of Artificial Sequence: Synthetic primer
gctgaagggcatcgacttcaagg

SEQ ID NO: 137 - DNA, 23 bp, Artificial Sequence
  Description of Artificial Sequence: Synthetic primer
cctcgaacttcacctcggcgcgg

SEQ ID NO: 138 - DNA, 23 bp, Artificial Sequence
  Description of Artificial Sequence: Synthetic primer
caagttcagcgtgtccggcgagg

SEQ ID NO: 139 - DNA, 23 bp, Artificial Sequence
  Description of Artificial Sequence: Synthetic primer
gaccaggatgggcaccaccccgg

SEQ ID NO: 140 - DNA, 23 bp, Artificial Sequence
  Description of Artificial Sequence: Synthetic primer
aagttcagcgtgtccggcgaggg

SEQ ID NO: 141 - DNA, 23 bp, Artificial Sequence
  Description of Artificial Sequence: Synthetic primer
gaccaggatgggcaccaccccgg

SEQ ID NO: 142 - DNA, 23 bp, Artificial Sequence
  Description of Artificial Sequence: Synthetic primer
gaagggcatcgacttcaaggagg

SEQ ID NO: 143 - DNA, 23 bp, Artificial Sequence
  Description of Artificial Sequence: Synthetic primer
cctcgaacttcacctcggcgcgg

SEQ ID NO: 144 - DNA, 23 bp, Artificial Sequence
  Description of Artificial Sequence: Synthetic primer
caactacaagacccgcgccgagg

SEQ ID NO: 145 - DNA, 23 bp, Artificial Sequence
  Description of Artificial Sequence: Synthetic primer
ctggacgtagccttcgggcatgg

SEQ ID NO: 146 - DNA, 23 bp, Artificial Sequence
  Description of Artificial Sequence: Synthetic primer
ggagcgcaccatcttcttcaagg

SEQ ID NO: 147 - DNA, 23 bp, Artificial Sequence
  Description of Artificial Sequence: Synthetic primer
agaagtcgtgctgcttcatgtgg

SEQ ID NO: 148 - DNA, 23 bp, Artificial Sequence
  Description of Artificial Sequence: Synthetic primer
caagttcagcgtgtccggcgagg

SEQ ID NO: 149 - DNA, 23 bp, Artificial Sequence
  Description of Artificial Sequence: Synthetic primer
cgtcgccgtccagctcgaccagg

SEQ ID NO: 150 - DNA, 23 bp, Artificial Sequence
  Description of Artificial Sequence: Synthetic primer
catgcccgaaggctacgtccagg

SEQ ID NO: 151 - DNA, 23 bp, Artificial Sequence
  Description of Artificial Sequence: Synthetic primer
agaagtcgtgctgcttcatgtgg

SEQ ID NO: 152 - DNA, 23 bp, Artificial Sequence
  Description of Artificial Sequence: Synthetic primer
caactacaagacccgcgccgagg

SEQ ID NO: 153 - DNA, 23 bp, Artificial Sequence
  Description of Artificial Sequence: Synthetic primer
tgaagaagatggtgcgctcctgg

SEQ ID NO: 154 - DNA, 23 bp, Artificial Sequence
  Description of Artificial Sequence: Synthetic primer
ggtgaaccgcatcgagctgaagg

SEQ ID NO: 155 - DNA, 23 bp, Artificial Sequence
  Description of Artificial Sequence: Synthetic primer
cctcgaacttcacctcggcgcgg

SEQ ID NO: 156 - DNA, 23 bp, Artificial Sequence
  Description of Artificial Sequence: Synthetic primer
ttcaagtccgccatgcccgaagg

SEQ ID NO: 157 - DNA, 23 bp, Artificial Sequence
  Description of Artificial Sequence: Synthetic primer
gcttcatgtggtcggggtagcgg

SEQ ID NO: 158 - DNA, 23 bp, Artificial Sequence
  Description of Artificial Sequence: Synthetic primer
ccgcgccgaggtgaagttcgagg

SEQ ID NO: 159 - DNA, 23 bp, Artificial Sequence
  Description of Artificial Sequence: Synthetic primer
gccgtcgtccttgaagaagatgg

SEQ ID NO: 160 - DNA, 23 bp, Artificial Sequence
  Description of Artificial Sequence: Synthetic primer
ggtgaaccgcatcgagctgaagg

SEQ ID NO: 161 - DNA, 23 bp, Artificial Sequence
  Description of Artificial Sequence: Synthetic primer
ctcgaacttcacctcggcgcggg

SEQ ID NO: 162 - DNA, 23 bp, Artificial Sequence
  Description of Artificial Sequence: Synthetic primer
gtgaaccgcatcgagctgaaggg

SEQ ID NO: 163 - DNA, 23 bp, Artificial Sequence
  Description of Artificial Sequence: Synthetic primer
cctcgaacttcacctcggcgcgg

SEQ ID NO: 164 - DNA, 23 bp, Artificial Sequence
  Description of Artificial Sequence: Synthetic primer
caagatccgccacaacatcgagg

SEQ ID NO: 165 - DNA, 23 bp, Artificial Sequence
  Description of Artificial Sequence: Synthetic primer
gatgccgttcttctgcttgtcgg

SEQ ID NO: 166 - DNA, 23 bp, Artificial Sequence
  Description of Artificial Sequence: Synthetic primer
gtgaaccgcatcgagctgaaggg

SEQ ID NO: 167 - DNA, 23 bp, Artificial Sequence
  Description of Artificial Sequence: Synthetic primer
ctcgaacttcacctcggcgcggg

SEQ ID NO: 168 - DNA, 23 bp, Artificial Sequence
  Description of Artificial Sequence: Synthetic primer
caaggaggacggcaacatcctgg

SEQ ID NO: 169 - DNA, 23 bp, Artificial Sequence
  Description of Artificial Sequence: Synthetic primer
tcagctcgatgcggttcaccagg

SEQ ID NO: 170 - DNA, 23 bp, Artificial Sequence
  Description of Artificial Sequence: Synthetic primer
catgcccgaaggctacgtccagg

SEQ ID NO: 171 - DNA, 23 bp, Artificial Sequence
  Description of Artificial Sequence: Synthetic primer
gtcgtgctgcttcatgtggtcgg

SEQ ID NO: 172 - DNA, 23 bp, Artificial Sequence
  Description of Artificial Sequence: Synthetic primer
caaggaggacggcaacatcctgg

SEQ ID NO: 173 - DNA, 23 bp, Artificial Sequence
  Description of Artificial Sequence: Synthetic primer
cagctcgatgcggttcaccaggg

SEQ ID NO: 174 - DNA, 23 bp, Artificial Sequence
  Description of Artificial Sequence: Synthetic primer
aaggaggacggcaacatcctggg

SEQ ID NO: 175 - DNA, 23 bp, Artificial Sequence
  Description of Artificial Sequence: Synthetic primer
tcagctcgatgcggttcaccagg

SEQ ID NO: 176 - DNA, 23 bp, Artificial Sequence
  Description of Artificial Sequence: Synthetic primer
aagttcagcgtgtccggcgaggg

SEQ ID NO: 177 - DNA, 23 bp, Artificial Sequence
  Description of Artificial Sequence: Synthetic primer
gccgtccagctcgaccaggatgg

SEQ ID NO: 178 - DNA, 23 bp, Artificial Sequence
  Description of Artificial Sequence: Synthetic primer
catgcccgaaggctacgtccagg

SEQ ID NO: 179 - DNA, 23 bp, Artificial Sequence
  Description of Artificial Sequence: Synthetic primer
tcgtgctgcttcatgtggtcggg

SEQ ID NO: 180 - DNA, 23 bp, Artificial Sequence
  Description of Artificial Sequence: Synthetic primer
aaggaggacggcaacatcctggg

SEQ ID NO: 181 - DNA, 23 bp, Artificial Sequence
  Description of Artificial Sequence: Synthetic primer
cagctcgatgcggttcaccaggg

SEQ ID NO: 182 - DNA, 23 bp, Artificial Sequence
  Description of Artificial Sequence: Synthetic primer
aggaggacggcaacatcctgggg

SEQ ID NO: 183 - DNA, 23 bp, Artificial Sequence
  Description of Artificial Sequence: Synthetic primer
tcagctcgatgcggttcaccagg

SEQ ID NO: 184 - DNA, 23 bp, Artificial Sequence
  Description of Artificial Sequence: Synthetic primer
atccgccacaacatcgaggacgg

SEQ ID NO: 185 - DNA, 23 bp, Artificial Sequence
  Description of Artificial Sequence: Synthetic primer
gatgccgttcttctgcttgtcgg

SEQ ID NO: 186 - DNA, 23 bp, Artificial Sequence
  Description of Artificial Sequence: Synthetic primer
cagcgtgtccggcgagggcgagg

SEQ ID NO: 187 - DNA, 23 bp, Artificial Sequence
  Description of Artificial Sequence: Synthetic primer
cgtcgccgtccagctcgaccagg

SEQ ID NO: 188 - DNA, 23 bp, Artificial Sequence
  Description of Artificial Sequence: Synthetic primer
ccggcaagctgcccgtgccctgg

SEQ ID NO: 189 - DNA, 23 bp, Artificial Sequence
  Description of Artificial Sequence: Synthetic primer
cagggtcagcttgccgtaggtgg

SEQ ID NO: 190 - DNA, 23 bp, Artificial Sequence
  Description of Artificial Sequence: Synthetic primer
catgcccgaaggctacgtccagg

SEQ ID NO: 191 - DNA, 23 bp, Artificial Sequence
  Description of Artificial Sequence: Synthetic primer
cgtgctgcttcatgtggtcgggg

SEQ ID NO: 192 - DNA, 23 bp, Artificial Sequence
  Description of Artificial Sequence: Synthetic primer
aggaggacggcaacatcctgggg

SEQ ID NO: 193 - DNA, 23 bp, Artificial Sequence
  Description of Artificial Sequence: Synthetic primer
cagctcgatgcggttcaccaggg

SEQ ID NO: 194 - DNA, 23 bp, Artificial Sequence
  Description of Artificial Sequence: Synthetic primer
caacatcctggggcacaagctgg

SEQ ID NO: 195 - DNA, 23 bp, Artificial Sequence
  Description of Artificial Sequence: Synthetic primer
cgatgcccttcagctcgatgcgg

SEQ ID NO: 196 - DNA, 23 bp, Artificial Sequence
  Description of Artificial Sequence: Synthetic primer
gctgaagggcatcgacttcaagg

SEQ ID NO: 197 - DNA, 23 bp, Artificial Sequence
  Description of Artificial Sequence: Synthetic primer
gtcgccctcgaacttcacctcgg

SEQ ID NO: 198 - DNA, 23 bp, Artificial Sequence
  Description of Artificial Sequence: Synthetic primer
ccagaagtacgagcgccgcccgg

SEQ ID NO: 199 - DNA, 23 bp, Artificial Sequence
  Description of Artificial Sequence: Synthetic primer
tggcaggtgagtgaggctgcagg

SEQ ID NO: 200 - DNA, 62 bp, Artificial Sequence
  Description of Artificial Sequence: Synthetic RFN target site oligonucleotide
ccgggcggcgctcgtacttctggccactgggcgagcgtctggcaggtgagtgaggctgcagg

SEQ ID NO: 201 - DNA, 23 bp, Artificial Sequence
  Description of Artificial Sequence: Synthetic primer
gaatacccatctgtcagcttcgg

SEQ ID NO: 202 - DNA, 23 bp, Artificial Sequence
  Description of Artificial Sequence: Synthetic primer
ggcggaacctgagaggcgtaagg

SEQ ID NO: 203 - DNA, 62 bp, Artificial Sequence
  Description of Artificial Sequence: Synthetic RFN target site oligonucleotide
ccgaagctgacagatgggtattctttgacggggggtaggggcggaacctgagaggcgtaagg

SEQ ID NO: 204 - DNA, 23 bp, Artificial Sequence
  Description of Artificial Sequence: Synthetic primer
aatattcaagcagcaggcacagg

SEQ ID NO: 205 - DNA, 23 bp, Artificial Sequence
  Description of Artificial Sequence: Synthetic primer
ctcgcgcaggaggctgcagcggg

SEQ ID NO: 206 - DNA, 62 bp, Artificial Sequence
  Description of Artificial Sequence: Synthetic RFN target site oligonucleotide
cctgtgcctgctgcttgaatatttccgccttttagggtgctcgcgcaggaggctgcagcggg

SEQ ID NO: 207 - DNA, 23 bp, Artificial Sequence
  Description of Artificial Sequence: Synthetic primer
cccaaagcctggccagggagtgg

SEQ ID NO: 208 - DNA, 23 bp, Artificial Sequence
  Description of Artificial Sequence: Synthetic primer
gccccacagggcttgaagcccgg

SEQ ID NO: 209 - DNA, 62 bp, Artificial Sequence
  Description of Artificial Sequence: Synthetic RFN target site oligonucleotide
ccactccctggccaggctttggggaggcctggagtcatggccccacagggcttgaagcccgg

SEQ ID NO: 210 - DNA, 23 bp, Artificial Sequence
  Description of Artificial Sequence: Synthetic primer
ccctacttccgctttcaccttgg

SEQ ID NO: 211 - DNA, 23 bp, Artificial Sequence
  Description of Artificial Sequence: Synthetic primer
ggaatcccttctgcagcacctgg

SEQ ID NO: 212 - DNA, 62 bp, Artificial Sequence
  Description of Artificial Sequence: Synthetic RFN target site oligonucleotide
ccaaggtgaaagcggaagtagggccttcgcgcacctcatggaatcccttctgcagcacctgg

SEQ ID NO: 213 - DNA, 23 bp, Artificial Sequence
  Description of Artificial Sequence: Synthetic primer
cgctccagagccgtgcgaatggg

SEQ ID NO: 214 - DNA, 23 bp, Artificial Sequence
  Description of Artificial Sequence: Synthetic primer
tggaggcaagagggcggctttgg

SEQ ID NO: 215 - DNA, 62 bp, Artificial Sequence
  Description of Artificial Sequence: Synthetic RFN target site oligonucleotide
cccattcgcacggctctggagcggcggctgcacaaccagtggaggcaagagggcggctttgg

SEQ ID NO: 216 - DNA, 23 bp, Artificial Sequence
  Description of Artificial Sequence: Synthetic primer
cgaggagactggggactgtaggg

SEQ ID NO: 217 - DNA, 23 bp, Artificial Sequence
  Description of Artificial Sequence: Synthetic primer
ccagctgctgccttgcctccagg

SEQ ID NO: 218 - DNA, 62 bp, Artificial Sequence
  Description of Artificial Sequence: Synthetic RFN target site oligonucleotide
ccctacagtccccagcctcctcgtcccatgcctccgtctccagctgctgccttgcctccagg

SEQ ID NO: 219 - DNA, 23 bp, Artificial Sequence
  Description of Artificial Sequence: Synthetic primer
catagctactgattggtggtggg

SEQ ID NO: 220 - DNA, 23 bp, Artificial Sequence
  Description of Artificial Sequence: Synthetic primer
ccggcccctccccagtcaggggg

SEQ ID NO: 221 - DNA, 62 bp, Artificial Sequence
  Description of Artificial Sequence: Synthetic RFN target site oligonucleotide
cccaccaccaatcagtagctatggcgagccctgctgtctccggcccctccccagtcaggggg

SEQ ID NO: 222 - DNA, 23 bp, Artificial Sequence
  Description of Artificial Sequence: Synthetic primer
ggaaacgtctagatgctcaacgg

SEQ ID NO: 223 - DNA, 23 bp, Artificial Sequence
  Description of Artificial Sequence: Synthetic primer
caaaatgtcgttcgtggcagtgg

SEQ ID NO: 224 - DNA, 62 bp, Artificial Sequence
  Description of Artificial Sequence: Synthetic RFN target site oligonucleotide
ccgttgagcatctagacgtttccttggctcttctggcgccaaaatgtcgttcgtggcagggg

SEQ ID NO: 225 - DNA, 23 bp, Artificial Sequence
  Description of Artificial Sequence: Synthetic primer
ctgttgctggccatgccaagcgg

SEQ ID NO: 226 - DNA, 23 bp, Artificial Sequence
  Description of Artificial Sequence: Synthetic primer
cctgggggcgggcacctcaatgg

SEQ ID NO: 227 - DNA, 62 bp, Artificial Sequence
  Description of Artificial Sequence: Synthetic RFN target site oligonucleotide
ccgcttggcatggccagcaacagcagctcctgcccgacacctgggggcgggcacctcaatgg

SEQ ID NO: 228 - DNA, 23 bp, Artificial Sequence
  Description of Artificial Sequence: Synthetic primer
ttcggagcgaaaaccaagacagg

SEQ ID NO: 229 - DNA, 23 bp, Artificial Sequence
  Description of Artificial Sequence: Synthetic primer
gagtcccccgccttcagaagagg

SEQ ID NO: 230 - DNA, 62 bp, Artificial Sequence
  Description of Artificial Sequence: Synthetic RFN target site oligonucleotide
cctgtcttggttttcgctccgaaggtaaaagaaatcattgagtcccccgccttcagaagagg

SEQ ID NO: 231 - DNA, 23 bp, Artificial Sequence
  Description of Artificial Sequence: Synthetic primer
ggcccggtcgactccgggcccgg

SEQ ID NO: 232 - DNA, 23 bp, Artificial Sequence
  Description of Artificial Sequence: Synthetic primer
tgctgggaatcagcagtgtttgg

SEQ ID NO: 233 - DNA, 62 bp, Artificial Sequence
  Description of Artificial Sequence: Synthetic RFN target site oligonucleotide
ccgggcccggagtcgaccgggccgaggcggaggcgggcctgctgggaatcagcagtgtttgg

SEQ ID NO: 234 - DNA, 23 bp, Artificial Sequence
  Description of Artificial Sequence: Synthetic primer
gggtggggggagtttgctcctgg

SEQ ID NO: 235 - DNA, 23 bp, Artificial Sequence
  Description of Artificial Sequence: Synthetic primer
tccctctttagccagagccgggg

SEQ ID NO: 236 - DNA, 62 bp, Artificial Sequence
  Description of Artificial Sequence: Synthetic RFN target site oligonucleotide
ccaggagcaaactccccccaccccctttccaaagcccattccctctttagccagagccgggg

SEQ ID NO: 237 - DNA, 23 bp, Artificial Sequence
  Description of Artificial Sequence: Synthetic primer
gccgccggccggggaggaggtgg

SEQ ID NO: 238 - DNA, 23 bp, Artificial Sequence
  Description of Artificial Sequence: Synthetic primer
ggcgagccgcgggcaggggccgg

SEQ ID NO: 239 - DNA, 62 bp, Artificial Sequence
  Description of Artificial Sequence: Synthetic RFN target site oligonucleotide
ccacctcctccccggccggcggcggacagtggacgcggcggcgagccgcgggcaggggccgg

SEQ ID NO: 240 - DNA, 23 bp, Artificial Sequence
  Description of Artificial Sequence: Synthetic primer
ccgtctgcacaccccggctctgg

SEQ ID NO: 241 - DNA, 23 bp, Artificial Sequence
  Description of Artificial Sequence: Synthetic primer
ctcggccaccacagggaagctgg

SEQ ID NO: 242 - DNA, 62 bp, Artificial Sequence
  Description of Artificial Sequence: Synthetic RFN target site oligonucleotide
ccagagccggggtgtgcagacggcagtcactagggggcgctcggccaccacagggaagctgg

SEQ ID NO: 243 - DNA, 20 bp, Artificial Sequence
  Description of Artificial Sequence: Synthetic primer
ggctgtgggaagccagcaac

SEQ ID NO: 244 - DNA, 20 bp, Artificial Sequence
  Description of Artificial Sequence: Synthetic primer
aagccaggggccaactggag

SEQ ID NO: 245 - DNA, 26 bp, Artificial Sequence
  Description of Artificial Sequence: Synthetic primer
gcgcgggaattacagataaattaaaa

SEQ ID NO: 246 - DNA, 25 bp, Artificial Sequence
  Description of Artificial Sequence: Synthetic primer
aggtcccatcctctcatacatacca

SEQ ID NO: 247 - DNA, 18 bp, Artificial Sequence
  Description of Artificial Sequence: Synthetic primer
accgccccttggcaccac

SEQ ID NO: 248 - DNA, 21 bp, Artificial Sequence
  Description of Artificial Sequence: Synthetic primer
cggagctcatctgcttcctgt

SEQ ID NO: 249 - DNA, 20 bp, Artificial Sequence
  Description of Artificial Sequence: Synthetic primer
ggagcagctggtcagagggg

SEQ ID NO: 250 - DNA, 20 bp, Artificial Sequence
  Description of Artificial Sequence: Synthetic primer
gggaagggggacactgggga

SEQ ID NO: 251 - DNA, 23 bp, Artificial Sequence
  Description of Artificial Sequence: Synthetic primer
gccctacatctgctctccctcca

SEQ ID NO: 252 - DNA, 20 bp, Artificial Sequence
  Description of Artificial Sequence: Synthetic primer
gggccgggaaagagttgctg

SEQ ID NO: 253 - DNA, 23 bp, Artificial Sequence
  Description of Artificial Sequence: Synthetic primer
gccctacatctgctctccctcca

SEQ ID NO: 254 - DNA, 20 bp, Artificial Sequence
  Description of Artificial Sequence: Synthetic primer
gggccgggaaagagttgctg

SEQ ID NO: 255 - DNA, 20 bp, Artificial Sequence
  Description of Artificial Sequence: Synthetic primer
ggggagggaggctccaggtt

SEQ ID NO: 256 - DNA, 20 bp, Artificial Sequence
  Description of Artificial Sequence: Synthetic primer
ggcacaatggctcccaagca

SEQ ID NO: 257 - DNA, 21 bp, Artificial Sequence
  Description of Artificial Sequence: Synthetic primer
ccttacccctcccctcactca

SEQ ID NO: 258 - DNA, 20 bp, Artificial Sequence
  Description of Artificial Sequence: Synthetic primer
agaagggcgggccagacagt

SEQ ID NO: 259 - DNA, 28 bp, Artificial Sequence
  Description of Artificial Sequence: Synthetic primer
atatccttctaggtagcgggcagtagcc

SEQ ID NO: 260 - DNA, 20 bp, Artificial Sequence
  Description of Artificial Sequence: Synthetic primer
tctcgggggagagcggtaaa

SEQ ID NO: 261 - DNA, 21 bp, Artificial Sequence
  Description of Artificial Sequence: Synthetic primer
cccaggaaaagtgccagctca

SEQ ID NO: 262 - DNA, 20 bp, Artificial Sequence
  Description of Artificial Sequence: Synthetic primer
tgatggtcaccccaactgga

SEQ ID NO: 263 - DNA, 19 bp, Artificial Sequence
  Description of Artificial Sequence: Synthetic primer
aaggcggcgctggcttttt

SEQ ID NO: 264 - DNA, 24 bp, Artificial Sequence
  Description of Artificial Sequence: Synthetic primer
ccagcacaacttactcgcacttga

SEQ ID NO: 265 - DNA, 20 bp, Artificial Sequence
  Description of Artificial Sequence: Synthetic primer
gggatgcagggacggtcaag

SEQ ID NO: 266 - DNA, 21 bp, Artificial Sequence
  Description of Artificial Sequence: Synthetic primer
gccgccccatccctagagaaa

SEQ ID NO: 267 - DNA, 20 bp, Artificial Sequence
  Description of Artificial Sequence: Synthetic primer
tccagatggcacattgtcag

SEQ ID NO: 268 - DNA, 20 bp, Artificial Sequence
  Description of Artificial Sequence: Synthetic primer
agggagcaggaaagtgaggt

SEQ ID NO: 269 - DNA, 22 bp, Artificial Sequence
  Description of Artificial Sequence: Synthetic primer
agagaagtcgaggaagagagag

SEQ ID NO: 270 - DNA, 22 bp, Artificial Sequence
  Description of Artificial Sequence: Synthetic primer
cagcagaaagttcatggtttcg

SEQ ID NO: 271 - DNA, 20 bp, Artificial Sequence
  Description of Artificial Sequence: Synthetic primer
tccagatggcacattgtcag

SEQ ID NO: 272 - DNA, 20 bp, Artificial Sequence
  Description of Artificial Sequence: Synthetic primer
agggagcaggaaagtgaggt

SEQ ID NO: 273 - DNA, 20 bp, Artificial Sequence
  Description of Artificial Sequence: Synthetic primer
cgatggctcccaagaaacgc

SEQ ID NO: 274 - DNA, 20 bp, Artificial Sequence
  Description of Artificial Sequence: Synthetic primer
gcaggtagaatgcacagccg

SEQ ID NO: 275 - DNA, 20 bp, Artificial Sequence
  Description of Artificial Sequence: Synthetic primer
gcccagagtcaaggaacacg

SEQ ID NO: 276 - DNA, 20 bp, Artificial Sequence
  Description of Artificial Sequence: Synthetic primer
aggtagtgcttgagaccgcc

SEQ ID NO: 277 - DNA, 20 bp, Artificial Sequence
  Description of Artificial Sequence: Synthetic primer
catccatcggcgctttggtc

SEQ ID NO: 278 - DNA, 20 bp, Artificial Sequence
  Description of Artificial Sequence: Synthetic primer
ccgggaaagagttgctgcac

SEQ ID NO: 279 - DNA, 20 bp, Artificial Sequence
  Description of Artificial Sequence: Synthetic primer
ctccccgtctgcagtccatc

SEQ ID NO: 280 - DNA, 20 bp, Artificial Sequence
  Description of Artificial Sequence: Synthetic primer
cctgcagggacatgtggtga

SEQ ID NO: 281 - DNA, 20 bp, Artificial Sequence
  Description of Artificial Sequence: Synthetic primer
tagggctagaggggtgaggc

SEQ ID NO: 282 - DNA, 20 bp, Artificial Sequence
  Description of Artificial Sequence: Synthetic primer
ccgaggtgaaacaagctgcc

SEQ ID NO: 283 - DNA, 20 bp, Artificial Sequence
  Description of Artificial Sequence: Synthetic primer
atgagggctccagatggcac

SEQ ID NO: 284 - DNA, 20 bp, Artificial Sequence
  Description of Artificial Sequence: Synthetic primer
ttcacccagcttccctgtgg

SEQ ID NO: 285 - DNA, 1752 bp, Planomicrobium okeanokoites
atgtttttgagtatggtttctaaaataagaactttcggttgggttcaaaatccaggtaaatttgagaatttaaaacgagtagttcaagtatttgatagaaattctaaagtacataatgaagtgaaaaatataaagataccaaccctagtcaaagaaagtaagatccaaaaagaactagttgctattatgaatcaacatgatttgatttatacatataaagagttagtaggaacaggaacttcaatacgttcagaagcaccatgcgatgcaattattcaagcaacaatagcagatcaaggaaataaaaaaggctatatcgataattggtcatctgacggttttttgcgttgggcacatgctttaggatttattgaatatataaataaaagtgattcttttgtaataactgatgttggacttgcttactctaaatcagctgacggcagcgccattgaaaaagagattttgattgaagcgatatcatcttatcctccagcgattcgtattttaactttgctagaagatggacaacatttgacaaagtttgatcttggcaagaatttaggttttagtggagaaagtggatttacttctctaccggaaggaattcttttagatactctagctaatgctatgcctaaagataaaggcgaaattcgtaataattgggaaggatcttcagataagtacgcaagaatgataggtggttggctggataaactaggattagtaaagcaaggaaaaaaagaatttatcattcctactttgggtaagccggacaataaagagtttatatcccacgcttttaaaattactggagaaggtttgaaagtactgcgtcgagcaaaaggctctacaaaatttacacgtgtacctaaaagagtatattgggaaatgcttgctacaaacctaaccgataaagagtatgtaagaacaagaagagctttgattttagaaatattaatcaaagctggatcattaaaaatagaacaaatacaagacaacttgaagaaattaggatttgatgaagttatagaaactattgaaaatgatatcaaaggcttaattaacacaggtatatttatagaaatcaaagggcgattttatcaattgaaagaccatattcttcaatttgtaatacctaatcgtggtgtgactaagcaactagtcaaaagtgaactggaggagaagaaatctgaacttcgtcataaattgaaatatgtgcctcatgaatatattgaattaattgaaattgccagaaattccactcaggatagaattcttgaaatgaaggtaatggaattttttatgaaagtttatggatatagaggtaaacatttgggtggatcaaggaaaccggacggagcaatttatactgtcggatctcctattgattacggtgtgatcgtggatactaaagcttatagcggaggttataatctgccaattggccaagcagatgaaatgcaacgatatgtcgaagaaaatcaaacacgaaacaaacatatcaaccctaatgaatggtggaaagtctatccatcttctgtaacggaatttaagtttttatttgtgagtggtcactttaaaggaaactacaaagctcagcttacacgattaaatcatatcactaattgtaatggagctgttcttagtgtagaagagcttttaattggtggagaaatgattaaagccggcacattaaccttagaggaagtgagacggaaatttaataacggcgagataaacttttaa

SEQ ID NO: 286 - DNA, 23 bp, Artificial Sequence
  Description of Artificial Sequence: Synthetic target binding site oligonucleotide
ggtgagtgagtgtgtgcgtgtgg

SEQ ID NO: 287 - DNA, 18 bp, Artificial Sequence
  Description of Artificial Sequence: Synthetic target binding site oligonucleotide
gggcgatgccacctacgg

SEQ ID NO: 288 - DNA, 20 bp, Artificial Sequence
  Description of Artificial Sequence: Synthetic target binding site oligonucleotide
gagggcgatgccacctacgg

SEQ ID NO: 289 - DNA, 22 bp, Artificial Sequence
  Description of Artificial Sequence: Synthetic target binding site oligonucleotide
gcgagggcgatgccacctacgg

SEQ ID NO: 290 - DNA, 23 bp, Artificial Sequence
  Description of Artificial Sequence: Synthetic target binding site oligonucleotide
ggcgagggcgatgccacctacgg

SEQ ID NO: 291 - DNA, 24 bp, Artificial Sequence
  Description of Artificial Sequence: Synthetic target binding site oligonucleotide
gggcgagggcgatgccacctacgg

SEQ ID NO: 292 - DNA, 26 bp, Artificial Sequence
  Description of Artificial Sequence: Synthetic target binding site oligonucleotide
gagggcgagggcgatgccacctacgg

SEQ ID NO: 293 - DNA, 28 bp, Artificial Sequence
  Description of Artificial Sequence: Synthetic target binding site oligonucleotide
gcgcgggcgagggcgatgccacctacgg

SEQ ID NO: 294 - DNA, 21 bp, Artificial Sequence
  Description of Artificial Sequence: Synthetic target binding site oligonucleotide
gcacgggcagcttgccggtgg

SEQ ID NO: 295 - DNA, 23 bp, Artificial Sequence
  Description of Artificial Sequence: Synthetic target binding site oligonucleotide
gggcacgggcagcttgccggtgg

SEQ ID NO: 296 - DNA, 20 bp, Artificial Sequence
  Description of Artificial Sequence: Synthetic target binding site oligonucleotide
gccgttcttctgcttgtcgg

SEQ ID NO: 297 - DNA, 23 bp, Artificial Sequence
  Description of Artificial Sequence: Synthetic target binding site oligonucleotide
gatgccgttcttctgcttgtcgg

SEQ ID NO: 298 - DNA, 19 bp, Artificial Sequence
  Description of Artificial Sequence: Synthetic target binding site oligonucleotide
gtgcagatgaacttcaggg

SEQ ID NO: 299 - DNA, 20 bp, Artificial Sequence
  Description of Artificial Sequence: Synthetic target binding site oligonucleotide
ggtgcagatgaacttcaggg

SEQ ID NO: 300 - DNA, 23 bp, Artificial Sequence
  Description of Artificial Sequence: Synthetic target binding site oligonucleotide
ggtggtgcagatgaacttcaggg

SEQ ID NO: 301 - DNA, 19 bp, Artificial Sequence
  Description of Artificial Sequence: Synthetic target binding site oligonucleotide
gaggagctgttcaccgggg

SEQ ID NO: 302 - DNA, 21 bp, Artificial Sequence
  Description of Artificial Sequence: Synthetic target binding site oligonucleotide
gcgaggagctgttcaccgggg

SEQ ID NO: 303 - DNA, 23 bp, Artificial Sequence
  Description of Artificial Sequence: Synthetic target binding site oligonucleotide
gggcgaggagctgttcaccgggg

SEQ ID NO: 304 - DNA, 21 bp, Artificial Sequence
  Description of Artificial Sequence: Synthetic target binding site oligonucleotide
gtggggggagtttgctcctgg

SEQ ID NO: 305 - DNA, 23 bp, Artificial Sequence
  Description of Artificial Sequence: Synthetic target binding site oligonucleotide
gggtggggggagtttgctcctgg

SEQ ID NO: 306 - DNA, 20 bp, Artificial Sequence
  Description of Artificial Sequence: Synthetic target binding site oligonucleotide
gagtgagtgtgtgcgtgtgg

SEQ ID NO: 307 - DNA, 23 bp, Artificial Sequence
  Description of Artificial Sequence: Synthetic target binding site oligonucleotide
ggtgagtgagtgtgtgcgtgtgg

SEQ ID NO: 308 - DNA, 21 bp, Artificial Sequence
  Description of Artificial Sequence: Synthetic target binding site oligonucleotide
gtccgagcagaagaagaaggg

SEQ ID NO: 309 - DNA, 23 bp, Artificial Sequence
  Description of Artificial Sequence: Synthetic target binding site oligonucleotide
gagtccgagcagaagaagaaggg

SEQ ID NO: 310 - DNA, 20 bp, Artificial Sequence
  Description of Artificial Sequence: Synthetic target binding site oligonucleotide
gatgtagtgtttccacaggg

SEQ ID NO: 311 - DNA, 23 bp, Artificial Sequence
  Description of Artificial Sequence: Synthetic target binding site oligonucleotide
gcagatgtagtgtttccacaggg

SEQ ID NO: 312 - DNA, 67 bp, Homo sapiens
gaagctggaggaggaagggcctgagtccgagcagaagaagaagggctcccatcacatcaaccggtgg

SEQ ID NO: 313 - DNA, 15 bp, Artificial Sequence
  Description of Artificial Sequence: Synthetic oligonucleotide
gaagctggaggagga

SEQ ID NO: 314 - DNA, 11 bp, Artificial Sequence
  Description of Artificial Sequence: Synthetic oligonucleotide
tcaaccggtgg

SEQ ID NO: 315 - DNA, 18 bp, Artificial Sequence
  Description of Artificial Sequence: Synthetic oligonucleotide
gaagctggaggaggaagg

SEQ ID NO: 316 - DNA, 25 bp, Artificial Sequence
  Description of Artificial Sequence: Synthetic oligonucleotide
gggctcccatcacatcaaccggtgg

SEQ ID NO: 317 - DNA, 24 bp, Artificial Sequence
  Description of Artificial Sequence: Synthetic oligonucleotide
gaagctggaggaggaagggcctga

SEQ ID NO: 318 - DNA, 14 bp, Artificial Sequence
  Description of Artificial Sequence: Synthetic oligonucleotide
gaagctggaggagg

SEQ ID NO: 319 - DNA, 39 bp, Artificial Sequence
  Description of Artificial Sequence: Synthetic oligonucleotide
gaagctggaggaggaagggcccatcacatcaaccggtgg

SEQ ID NO: 320 - DNA, 40 bp, Artificial Sequence
  Description of Artificial Sequence: Synthetic oligonucleotide
gaagctggaggaggaagggctcgcacacatcaaccggtgg

SEQ ID NO: 321 - DNA, 42 bp, Artificial Sequence
  Description of Artificial Sequence: Synthetic oligonucleotide
gaagctggaggaggaagggccttccatcacatcaaccggtgg

SEQ ID NO: 322 - DNA, 46 bp, Artificial Sequence
  Description of Artificial Sequence: Synthetic oligonucleotide
gaagctggaggaggaagggcctgagtcccatcacatcaaccggtgg

SEQ ID NO: 323 - DNA, 52 bp, Artificial Sequence
  Description of Artificial Sequence: Synthetic oligonucleotide
gaagctggaggaggaagggcctgagtccgagtcccatcacatcaaccggtgg

SEQ ID NO: 324 - DNA, 58 bp, Artificial Sequence
  Description of Artificial Sequence: Synthetic oligonucleotide
gaagctggaggaggaagggcctgagtccgagcagaagtcccatcacatcaaccggtgg

SEQ ID NO: 325 - DNA, 59 bp, Artificial Sequence
  Description of Artificial Sequence: Synthetic oligonucleotide
gaagctggaggaggaagggcctgagtcctgccgtttgtagccatcacatcaaccggtgg

SEQ ID NO: 326 - DNA, 61 bp, Artificial Sequence
  Description of Artificial Sequence: Synthetic oligonucleotide
gaagctggaggaggaagggcctgagtccgagcagaagagctcccatcacatcaaccggtgg

SEQ ID NO: 327 - DNA, 61 bp, Artificial Sequence
  Description of Artificial Sequence: Synthetic oligonucleotide
gaagctggaggaggaagggcctgagtccgagcagaagaactcccatcacatcaaccggtgg

SEQ ID NO: 328 - DNA, 64 bp, Artificial Sequence
  Description of Artificial Sequence: Synthetic oligonucleotide
gaagctggaggaggaagggcctgagtccgagcagaagaagggctcccatcacatcaaccggtgg

SEQ ID NO: 329 - DNA, 65 bp, Artificial Sequence
  Description of Artificial Sequence: Synthetic oligonucleotide
gaagctggaggaggaagggcctgagtccgagcagaagaaagggctcccatcacatcaaccggtgg

SEQ ID NO: 330 - DNA, 67 bp, Artificial Sequence
  Description of Artificial Sequence: Synthetic oligonucleotide
gaagctggaggaggaagggcctgagtccgagcagaagaacagaagggctcccatcacatcaaccggt

SEQ ID NO: 331 - DNA, 67 bp, Homo sapiens; identical to SEQ ID NO: 312

SEQ ID NO: 332 - DNA, 31 bp, Artificial Sequence
  Description of Artificial Sequence: Synthetic oligonucleotide
gaagctggaggaggaagggcctgagtccgag

SEQ ID NO: 333 - DNA, 11 bp, Artificial Sequence
  Description of Artificial Sequence: Synthetic oligonucleotide
gaagctggagg

SEQ ID NO: 334 - DNA, 11 bp, Artificial Sequence
  Description of Artificial Sequence: Synthetic oligonucleotide
gaagctggagg

SEQ ID NO: 335 - DNA, 28 bp, Artificial Sequence
  Description of Artificial Sequence: Synthetic oligonucleotide
gaagctggaggaggaagggcctgagtgg

SEQ ID NO: 336 - DNA, 41 bp, Artificial Sequence
  Description of Artificial Sequence: Synthetic oligonucleotide
gaagctggaggaggaagggctcccatcacatcaaccggtgg

SEQ ID NO: 337 - DNA, 45 bp, Artificial Sequence
  Description of Artificial Sequence: Synthetic oligonucleotide
gaagctggaggaggaagggcctgagtccatcacatcaaccggtgg

SEQ ID NO: 338 - DNA, 46 bp, Artificial Sequence; identical to SEQ ID NO: 322
  Description of Artificial Sequence: Synthetic oligonucleotide

SEQ ID NO: 339 - DNA, 49 bp, Artificial Sequence
  Description of Artificial Sequence: Synthetic oligonucleotide
gaagctggaggaggaagggcctgagtccgagcatcacatcaaccggtgg

SEQ ID NO: 340 - DNA, 53 bp, Artificial Sequence
  Description of Artificial Sequence: Synthetic oligonucleotide
gaagctggaggaggaagggcctgagtccgagctcccatcacatcaaccggtgg

SEQ ID NO: 341 - DNA, 61 bp, Artificial Sequence
  Description of Artificial Sequence: Synthetic oligonucleotide
gaagctggaggaggaagggcctgagtccgagcagaagggctcccatcacatcaaccggtgg

SEQ ID NO: 342 - DNA, 64 bp, Artificial Sequence; identical to SEQ ID NO: 328
  Description of Artificial Sequence: Synthetic oligonucleotide

SEQ ID NO: 343 - DNA, 65 bp, Artificial Sequence
  Description of Artificial Sequence: Synthetic oligonucleotide
gaagctggaggaggaagggcctgagtccgagcagaaagaagggctcccatcacatcaaccggtgg

SEQ ID NO: 344 - DNA, 67 bp, Artificial Sequence; identical to SEQ ID NO: 330
  Description of Artificial Sequence: Synthetic oligonucleotide

SEQ ID NO: 345 - DNA, 187 bp, Aequorea victoria
tcgtgaccaccctgacctacggcgtgcagtgcttcagccgctaccccgaccacatgaagcagcacgacttcttcaagtccgccatgcccgaaggctacgtccaggagcgcaccatcttcttcaaggagacggcaactacaagacccgcgccgaggtgaagttcgagggcgacaccctggtgaaccgc

SEQ ID NO: 346 - DNA, 184 bp, Artificial Sequence
  Description of Artificial Sequence: Synthetic polynucleotide
tcgtgaccaccctgacctacgtgcagtgcttcagccgctaccccgaccacatgaagcagcacgacttcttcaagtccgccatgcccgaaggctacgtccaggagcgcaccatcttcttcaaggacgacggcaactacaagacccgcgcgaggtgaagttcgagggcgacaccctggtgaaccgc

SEQ ID NO: 347 - DNA, 159 bp, Artificial Sequence
  Description of Artificial Sequence: Synthetic polynucleotide
tcgtgaccaccctgacctcagccgctaccccgaccacatgaagcagcacgacttcttcaagtccgccatgcccgaaggctacgtccaggagcgcaccatcttcttcaaggacgacggcaactacaagacccgcgccgaggcgacaccctggtgaaccgc

SEQ ID NO: 348 - DNA, 154 bp, Artificial Sequence
  Description of Artificial Sequence: Synthetic polynucleotide
tcgtgaccaccctgacctacggcgtgcagtgcttcagccgctaccccgaccacatgaagcagcacgacttcttcaagtccgccatgcccgaaggctacgtccaggagcgcaccatcttcttcaaggagacggcaactacaccctggtgaaccgc

SEQ ID NO: 349 - DNA, 181 bp, Artificial Sequence
  Description of Artificial Sequence: Synthetic polynucleotide
tcgtgaccaccctgaccgtgcagtgcttcagccgctaccccgaccacatgaagcagcacgacttcttcaagtccgccatgcccgaaggctacgtccaggagcgcaccatcttcttcaaggacgacggcaactacaagacccgcgcgagggtcttgttcgagggcgacaccctggtgaaccg

SEQ ID NO: 350 - DNA, 53 bp, Artificial Sequence
  Description of Artificial Sequence: Synthetic oligonucleotide
tcgtgaccaccctgacctacgtgaagttcgagggcgacaccctggtgaaccgc

SEQ ID NO: 351 - DNA, 187 bp, Artificial Sequence
  Description of Artificial Sequence: Synthetic polynucleotide
tcgtgaccaccctgacctacgcctcggcgcgggtcttgtagttgccgtcgtccttgaagaagatggtgcgctcctggacgtagccttcgggcatggcggacttgaagaagtcgtgctgcttcatgtgtcggggtagcggctgaagcactgcacgctgaagttcgagggcgacaccctggtgaaccgc

SEQ ID NO: 352 - DNA, 146 bp, Artificial Sequence
  Description of Artificial Sequence: Synthetic polynucleotide
tcggcgcgggtcttgtagttgccgtcgtccttgaagaagatggtgcgctcctggacgtagccttcgggcatggcggacttgaagaagtcgtgctgcttcatgtggtcggggtagcggctgaagcactgcacaccctggtgaaccgc

SEQ ID NO: 353 - DNA, 41 bp, Artificial Sequence
  Description of Artificial Sequence: Synthetic oligonucleotide
tcgtgaccaccctgttcgagggcgacaccctggtgaaccgc

SEQ ID NO: 354 - DNA, 92 bp, Homo sapiens
caggagacgaagagcccgggcggcgctcgtacttctggccactgggcgagcgtctggcaggtgagtgaggctgcaggcattgacgtctcctc

SEQ ID NO: 355 - DNA, 92 bp, Artificial Sequence
  Description of Artificial Sequence: Synthetic oligonucleotide
caggagacgaagagcccgggcggcgctcgtacttctggccactggcgaagcgtctggcaggtgagtgaggctgcaggcattgacgtctcctc

SEQ ID NO: 356 - DNA, 80 bp, Artificial Sequence
  Description of Artificial Sequence: Synthetic oligonucleotide
caggagacgaagagcccgggcggcgctcgtacttctggcctctggcaggtgagtgaggctgcaggcattgacgtctcctc

SEQ ID NO: 357 - DNA, 80 bp, Artificial Sequence
  Description of Artificial Sequence: Synthetic oligonucleotide
caggagacgaagagcccgggcggcgctcgtacttctagcgtctggcaggtgagtgaggctgcaggcattgacgtctcctc

SEQ ID NO: 358 - DNA, 76 bp, Artificial Sequence
  Description of Artificial Sequence: Synthetic oligonucleotide
caggagacgaagagcccgggcggcgctcgtacttcgtctggcaggtgagtgaggctgcaggcattgacgtctcctc

SEQ ID NO: 359 - DNA, 75 bp, Artificial Sequence
  Description of Artificial Sequence: Synthetic oligonucleotide
caggagacgaagagcccgggcggcgctcgtacttctggccactgtgagtgaggctgcaggcattgacgtctcctc

SEQ ID NO: 360 - DNA, 73 bp, Artificial Sequence
  Description of Artificial Sequence: Synthetic oligonucleotide
caggagacgaagagcccgggcggcgctcgtacttctggcaggtgagtgaggctgcaggcattgacgtctcctc

SEQ ID NO: 361 - DNA, 69 bp, Artificial Sequence
  Description of Artificial Sequence: Synthetic oligonucleotide
caggagacgaagagcccgggcggcgctcgtctggcaggtgagtgaggctgcaggcattgacgtctcctc

SEQ ID NO: 362 - DNA, 58 bp, Artificial Sequence
  Description of Artificial Sequence: Synthetic oligonucleotide
caggagacgaagagcccgtctggcaggtgagtgaggctgcaggcattgacgtctcctc

SEQ ID NO: 363 - DNA, 46 bp, Artificial Sequence
  Description of Artificial Sequence: Synthetic oligonucleotide
accggcggcagcaggtgagtgaggctgcaggcattgacgtctcctc

SEQ ID NO: 364 - DNA, 92 bp, Homo sapiens
tgggagagtggatttccgaagctgacagatgggtattctttgagggggggtaggggcggaacctgagaggcgtaaggcgttgtgaaccctgg

SEQ ID NO: 365 - DNA, 86 bp, Artificial Sequence
  Description of Artificial Sequence: Synthetic oligonucleotide
tgggagagtggatttccgaagctgacagatgggtattctttgagtaggggcggaacctgagaggcgtaaggcgttgtgaaccctgg

SEQ ID NO: 366 - DNA, 84 bp, Artificial Sequence
  Description of Artificial Sequence: Synthetic oligonucleotide
tgggagagtggatttccgaagctgacagatgggtatggggggtaggggcggaacctgagaggcgtaaggcgttgtgaaccctgg

SEQ ID NO: 367 - DNA, 84 bp, Artificial Sequence
  Description of Artificial Sequence: Synthetic oligonucleotide
tgggagagtggatttccgaagctgacagatgggtattcttggtaggggcggaacctgagaggcgtaaggcgttgtgaaccctgg

SEQ ID NO: 368 - DNA, 82 bp, Artificial Sequence
  Description of Artificial Sequence: Synthetic oligonucleotide
tgggagagtggatttccgaagctgacagatgggtattctttgaggggggaacctgagaggcgtaaggcgttgtgaaccctgg

SEQ ID NO: 369 - DNA, 80 bp, Artificial Sequence
  Description of Artificial Sequence: Synthetic oligonucleotide
tgggagagtggatttccgaagctgacagatgggtattctttgggcggaacctgagaggcgtaaggcgttgtgaaccctgg

SEQ ID NO: 370 - DNA, 70 bp, Artificial Sequence
  Description of Artificial Sequence: Synthetic oligonucleotide
tgggagagtggatttccgaagctgacagatggggcggaacctgagaggcgtaaggcgttgtgaaccctgg

SEQ ID NO: 371 - DNA, 92 bp, Homo sapiens
caagctggactctggccactccctggccaggctttggggaggcctggagtcatggccccacagggcttgaagcccggggggccgccattgac

SEQ ID NO: 372 - DNA, 76 bp, Artificial Sequence
  Description of Artificial Sequence: Synthetic oligonucleotide
caagctggactctggccactccctggccaggctttatggccccacagggcttgaagcccggggggccgccattgac

SEQ ID NO: 373 - DNA, 92 bp, Homo sapiens
agagagtcgccgtctccaaggtgaaagcggaagtagggccttcgcgcacctcatggaatcccttctgcagcacctggatcgcttttccgagc

SEQ ID NO: 374 - DNA, 84 bp, Artificial Sequence
  Description of Artificial Sequence: Synthetic oligonucleotide
agagagtcgccgtctccaaggtgaaagcggaagtagcgcacctcatggaatcccttctgcagcacctggatcgcttttccgagc

SEQ ID NO: 375 - DNA, 83 bp, Artificial Sequence
  Description of Artificial Sequence: Synthetic oligonucleotide
agagagtcgccgtctccaaggtgaaagcggaagtagggccctcatggaatcccttctgcagcacctggatcgcttttccgagc

SEQ ID NO: 376 - DNA, 82 bp, Artificial Sequence
  Description of Artificial Sequence: Synthetic oligonucleotide
agagagtcgccgtctccaaggtgaaagcggaagtaggccctcatggaatcccttctgcagcacctggatcgcttttccgagc

SEQ ID NO: 377 - DNA, 82 bp, Artificial Sequence
  Description of Artificial Sequence: Synthetic oligonucleotide
agagagtcgccgtctccaaggtgaaagcggaagtagggcctcatggaatcccttctgcagcacctggatcgcttttccgagc

SEQ ID NO: 378 - DNA, 82 bp, Artificial Sequence
  Description of Artificial Sequence: Synthetic oligonucleotide
agagagtcgccgtctccaaggtgaaagcggaagtagcacctcatggaatcccttctgcagcacctggatcgcttttccgagc

SEQ ID NO: 379 - DNA, 81 bp, Artificial Sequence
  Description of Artificial Sequence: Synthetic oligonucleotide
agagagtcgccgtctccaaggtgaaagcggaaacgcacctcatggaatcccttctgcagcacctggatcgcttttccgagc

SEQ ID NO: 380 - DNA, 78 bp, Artificial Sequence
  Description of Artificial Sequence: Synthetic oligonucleotide
agagagtcgccgtctccaaggtgaaagcggaagtagggccttcgcgcattctgcagcacctggatcgcttttccgagc

SEQ ID NO: 381 - DNA, 77 bp, Artificial Sequence
  Description of Artificial Sequence: Synthetic oligonucleotide
agagagtcgccgtctccaaggtgaaagcggaagcctcatggaatcccttctgcagcacctggatcgcttttccgagc

SEQ ID NO: 382 - DNA, 61 bp, Artificial Sequence
  Description of Artificial Sequence: Synthetic oligonucleotide
agagagtcgccgtctccaagcatggaatcccttctgcagcacctggatcgcttttccgagc

SEQ ID NO: 383 - DNA, 92 bp, Homo sapiens
tttggtcggcatggccccattcgcacggctctggagcggcggctgcacaaccagtggaggcaagagggcggctttgggcggggtccagttcc

SEQ ID NO: 384 - DNA, 89 bp, Artificial Sequence
  Description of Artificial Sequence: Synthetic oligonucleotide
tttggtcggcatggccccattcgcacggctctggagcggcggcgcaaccagtggaggcaagagggcggctttgggcggggtccagttcc

SEQ ID NO: 385 - DNA, 88 bp, Artificial Sequence
  Description of Artificial Sequence: Synthetic oligonucleotide
tttggtcggcatggccccattcgcacggctctggagcggcggctaaccagtggaggcaagagggcggctttgggcggggtccagttcc

SEQ ID NO: 386 - DNA, 84 bp, Artificial Sequence
  Description of Artificial Sequence: Synthetic oligonucleotide
tttggtcggcatggccccattcgcacggctctggagcggcggccagtggaggcaagagggcggctttgggcggggtccagttcc

SEQ ID NO: 387 - DNA, 83 bp, Artificial Sequence
  Description of Artificial Sequence: Synthetic oligonucleotide
tttggtcggcatggccccattcgcacggctctggagcggcggctgtggaggcaagagggcggctttgggcggggtccagttcc

SEQ ID NO: 388 - DNA, 81 bp, Artificial Sequence
  Description of Artificial Sequence: Synthetic oligonucleotide
tttggtcggcatggccccattcgcacggctctggagcggcggctggaggcaagagggcggctttgggcggggtccagttcc

SEQ ID NO: 389 - DNA, 80 bp, Artificial Sequence
  Description of Artificial Sequence: Synthetic oligonucleotide
tttggtcggcatggccccattcgcacggctctggagcggcgggagaggcaagagggcggctttgggcggggtccagttcc

SEQ ID NO: 390 - DNA, 79 bp, Artificial Sequence
  Description of Artificial Sequence: Synthetic oligonucleotide
tttggtcggcatggccccattcgcacggctctggagcggcggcgaggcaagagggcggctttgggcggggtccagttcc

SEQ ID NO: 391 - DNA, 78 bp, Artificial Sequence
  Description of Artificial Sequence: Synthetic oligonucleotide
tttggtcggcatggccccattcgcacggctctggagcggcggctggcaagagggcggctttgggcggggtccagttcc

SEQ ID NO: 392 - DNA, 77 bp, Artificial Sequence
  Description of Artificial Sequence: Synthetic oligonucleotide
tttggtcggcatggccccattcgcacggctctggagcggcggcggcaagagggcggctttgggcggggtccagttcc

SEQ ID NO: 393 - DNA, 74 bp, Artificial Sequence
  Description of Artificial Sequence: Synthetic oligonucleotide
tttggtcggcatggccccattcgcacggctctggagtggaggcaagagggcggctttgggcggggtccagttcc

SEQ ID NO: 394 - DNA, 69 bp, Artificial Sequence
  Description of Artificial Sequence: Synthetic oligonucleotide
tttggtcggcatggccccattcgcacggctctggaggcaagagggcggctttgggcggggtccagttcc

SEQ ID NO: 395 - DNA, 26 bp, Artificial Sequence
  Description of Artificial Sequence: Synthetic oligonucleotide
tttggtcggcatggccccgtcactgt

SEQ ID NO: 396 - DNA, 260 bp, Artificial Sequence
  Description of Artificial Sequence: Synthetic polynucleotide
tttggtcggcatggccccattcgcacggctctggagcggcggcacactattgcaatgaaaataaatttcctttattagctagaagtgagatctgaaggggcttcatgatgtccccataatttttggcagagggaaaaagatctcagtggtatttgtgagccagggcattggccacaccagccaccaccttttgataggcagcctgcacctgaggagtgcgagtggaggcaagagggcggctttgggcggggtccagttcc

SEQ ID NO: 397 - DNA, 92 bp, Homo sapiens
gttcaactcgatgaccccaccaccaatcagtagctatggcgagccctgctgtctccggcccctccccagtcagggggcccccagtgtgggga

SEQ ID NO: 398 - DNA, 85 bp, Artificial Sequence
  Description of Artificial Sequence: Synthetic oligonucleotide
gttcaactcgatgaccccaccaccaatcagtagctatcctgctgtctccggcccctccccagtcagggggcccccagtgtgggga

SEQ ID NO: 399 - DNA, 79 bp, Artificial Sequence
  Description of Artificial Sequence: Synthetic oligonucleotide
gttcaactcgatgaccccaccaccaatcagtagctatgtctccggcccctccccagtcagggggcccccagtgtgggga

SEQ ID NO: 400 - DNA, 75 bp, Artificial Sequence
  Description of Artificial Sequence: Synthetic oligonucleotide
gttcaactcgatgaccccaccaccaatcagtagctatggcgagcccccccagtcagggggcccccagtgtgggga

SEQ ID NO: 401 - DNA, 74 bp, Artificial Sequence
  Description of Artificial Sequence: Synthetic oligonucleotide
gttcaactcgatgaccccaccaccaacctgctgtctccggcccctccccagtcagggggcccccagtgtgggga

SEQ ID NO: 402 - DNA, 92 bp, Homo sapiens
tggctgaaggcacttccgttgagcatctagacgtttccttggctcttctggcgccaaaatgtcgttcgtggcaggggttattcggcggctgg

SEQ ID NO: 403 - DNA, 83 bp, Artificial Sequence
  Description of Artificial Sequence: Synthetic oligonucleotide
tggctgaaggcacttccgttgagcatctagacgtttccttggcgccaaaatgtcgttcgtggcaggggttattcggcggctgg

SEQ ID NO: 404 - DNA, 76 bp, Artificial Sequence
  Description of Artificial Sequence: Synthetic oligonucleotide
tggctgaaggcacttccgttgagcatctattctggcgccaaaatgtcgttcgtggcaggggttattcggcggctgg

SEQ ID NO: 405 - DNA, 76 bp, Artificial Sequence
  Description of Artificial Sequence: Synthetic oligonucleotide
tggctgaaggcacttccgttgagcatctagacgtttccttggatgtcgttcgtggcaggggttattcggcggctgg

SEQ ID NO: 406 - DNA, 68 bp, Artificial Sequence
  Description of Artificial Sequence: Synthetic oligonucleotide
tggctgaaggcacttccgttgagcatctagacgtttgtcgttcgtggcaggggttattcggcggctgg

SEQ ID NO: 407 - DNA, 92 bp, Homo sapiens
cccttctgactgtggccgcttggcatggccagcaacagcagctcctgcccgacacctgggggcgggcacctcaatgggtacccggtgcctcc

SEQ ID NO: 408 - DNA, 86 bp, Artificial Sequence
  Description of Artificial Sequence: Synthetic oligonucleotide
cccttctgactgtggccgcttggcatggccagcaacacctgcccgacacctgggggcgggcacctcaatgggtacccggtgcctcc

SEQ ID NO: 409 - DNA, 85 bp, Artificial Sequence
  Description of Artificial Sequence: Synthetic oligonucleotide
cccttctgactgtggccgcttggcatggccagcaacactgcccgacacctgggggcgggcacctcaatgggtacccggtgcctcc

SEQ ID NO: 410 - DNA, 80 bp, Artificial Sequence
  Description of Artificial Sequence: Synthetic oligonucleotide
cccttctgactgtggccgcttggcatggccagcagcccgacacctgggggcgggcacctcaatgggtacccggtgcctcc

SEQ ID NO: 411 - DNA, 78 bp, Artificial Sequence
  Description of Artificial Sequence: Synthetic oligonucleotide
cccttctgactgtggccgcttggcatggccaggcccgacacctgggggcgggcacctcaatgggtacccggtgcctcc

SEQ ID NO: 412 - DNA, 92 bp, Homo sapiens
tcagaaatagggggtccaggagcaaactccccccaccccctttccaaagcccattccctctttagccagagccggggtgtgcagacggcagt

SEQ ID NO: 413 - DNA, 92 bp, Artificial Sequence
  Description of Artificial Sequence: Synthetic oligonucleotide
tcagaaatagggggtccaggagcaaactccccccaccccctttccaaaaagcccattccctctttagccagagccggggtgtgcagacggca

SEQ ID NO: 414 - DNA, 89 bp, Artificial Sequence
  Description of Artificial Sequence: Synthetic oligonucleotide
tcagaaatagggggtccaggagcaaactccccccaccccctttccgcccattccctctttagccagagccggggtgtgcagacggcagt

SEQ ID NO: 415 - DNA, 87 bp, Artificial Sequence
  Description of Artificial Sequence: Synthetic oligonucleotide
tcagaaatagggggtccaggagcaaactccccccacccccttagcccattccctctttagccagagccggggtgtgcagacggcagt

SEQ ID NO: 416 - DNA, 87 bp, Artificial Sequence
  Description of Artificial Sequence: Synthetic oligonucleotide
tcagaaatagggggtccaggagcaaactccccccacccccaaagcccattccctctttagccagagccggggtgtgcagacggcagt

SEQ ID NO: 417 - DNA, 86 bp, Artificial Sequence
  Description of Artificial Sequence: Synthetic oligonucleotide
tcagaaatagggggtccaggagcaaactccccccaccccaaagcccattccctctttagccagagccggggtgtgcagacggcagt

SEQ ID NO: 418 - DNA, 85 bp, Artificial Sequence
  Description of Artificial Sequence: Synthetic oligonucleotide
tcagaaatagggggtccaggagcaaactccccccaccccctttccattccctctttagccagagccggggtgtgcagacggcagt

SEQ ID NO: 419 - DNA, 84 bp, Artificial Sequence
  Description of Artificial Sequence: Synthetic oligonucleotide
tcagaaatagggggtccaggagcaaactccccccaccccctttcattccctctttagccagagccggggtgtgcagacggcagt

SEQ ID NO: 420 - DNA, 83 bp, Artificial Sequence
  Description of Artificial Sequence: Synthetic oligonucleotide
tcagaaatagggggtccaggagcaaactccccccacaaagcccattccctctttagccagagccggggtgtgcagacggcagt

SEQ ID NO: 421 - DNA, 78 bp, Artificial Sequence
  Description of Artificial Sequence: Synthetic oligonucleotide
tcagaaatagggggtccaggagcaaactccccccacccattccctctttagccagagccggggtgtgcagacggcagt

SEQ ID NO: 422 - DNA, 75 bp, Artificial Sequence
  Description of Artificial Sequence: Synthetic oligonucleotide
tcagaaatagggggtccaggagcaaaccaaagcccattccctctttagccagagccggggtgtgcagacggcagt

SEQ ID NO: 423 - DNA, 74 bp, Artificial Sequence
  Description of Artificial Sequence: Synthetic oligonucleotide
tcagaaatagggggtccaggagcaaactccccccaccccctctttagccagagccggggtgtgcagacggcagt

SEQ ID NO: 424 - DNA, 72 bp, Artificial Sequence
  Description of Artificial Sequence: Synthetic oligonucleotide
tcagaaatagggggtccaggagcaaactccccccaccccctttagccagagccggggtgtgcagacggcagt

SEQ ID NO: 425 - DNA, 68 bp, Artificial Sequence
  Description of Artificial Sequence: Synthetic oligonucleotide
tcagaaatagggggtccaggcaaagcccattccctctttagccagagccggggtgtgcagacggcagt

SEQ ID NO: 426 - DNA, 57 bp, Artificial Sequence
  Description of Artificial Sequence: Synthetic oligonucleotide
tcagaaatagggggtccaggagctctttagccagagccggggtgtgcagacggcagt

SEQ ID NO: 427 - DNA, 92 bp, Homo sapiens
ccccagccccagctaccacctcctccccggccggcggcggacagtggacgcggcggcgagccgcgggcaggggccggagcccgcgcccggag

SEQ ID NO: 428 - DNA, 84 bp, Artificial Sequence
  Description of Artificial Sequence: Synthetic oligonucleotide
ccccagccccagctaccacctcctccccggccggcgtggacgcggcggcgagccgcgggcaggggccggagcccgcgcccggag

SEQ ID NO: 429 - DNA, 79 bp, Artificial Sequence
  Description of Artificial Sequence: Synthetic oligonucleotide
ccccagccccagctaccacctcctccccggccggacgcggcggcgagccgcgggcaggggccggagcccgcgcccggag

SEQ ID NO: 430 - DNA, 79 bp, Artificial Sequence
  Description of Artificial Sequence: Synthetic oligonucleotide
ccccagccccagctaccacctcctccccggctggacgcggcggcgagccgcgggcaggggccggagcccgcgcccggag

SEQ ID NO: 431 - DNA, 76 bp, Artificial Sequence
  Description of Artificial Sequence: Synthetic oligonucleotide
ccccagccccagctaccacctcctccccggccggcggcggacagccgcgggcaggggccggagcccgcgcccggag

SEQ ID NO: 432 - DNA, 75 bp, Artificial Sequence
  Description of Artificial Sequence: Synthetic oligonucleotide
ccccagccccagctaccacctcctccccggacgcggcggcgagccgcgggcaggggccggagcccgcgcccggag

SEQ ID NO: 433 - DNA, 49 bp, Artificial Sequence
  Description of Artificial Sequence: Synthetic oligonucleotide
ccccagccccagctaccacctcctccccggccggagcccgcgcccgaag

SEQ ID NO: 434 - DNA, 63 bp, Artificial Sequence
  Description of Artificial Sequence: Synthetic oligonucleotide
ccccagccccagctaccacctcctccccggccggcggcggacagtggagggggtcggggctcg

SEQ ID NO: 435 - DNA, 36 bp, Artificial Sequence
  Description of Artificial Sequence: Synthetic oligonucleotide
ccccagccccagctaccacctcctccccggccggag

SEQ ID NO: 436 - DNA, 55 bp, Artificial Sequence
  Description of Artificial Sequence: Synthetic oligonucleotide
ccccagccccagctaccacctcctccccggccggcggcggggtggagggggtcgg

SEQ ID NO: 437 - DNA, 60 bp, Artificial Sequence
  Description of Artificial Sequence: Synthetic oligonucleotide
ccccagccccagctaccacctcctccccggccggcggcggacacacacgcggcgtcgcac

SEQ ID NO: 438 - DNA, 53 bp, Artificial Sequence
  Description of Artificial Sequence: Synthetic oligonucleotide
ccccagccccagctaccacctcctccccggccggcggcctgaaacttttcgtc

SEQ ID NO: 439 - DNA, 30 bp, Artificial Sequence
  Description of Artificial Sequence: Synthetic oligonucleotide
ccggagcgcggcgtggagggggtcggggct

SEQ ID NO: 440 - DNA, 92 bp, Homo sapiens
ccattccctctttagccagagccggggtgtgcagacggcagtcactagggggcgctcggccaccacagggaagctgggtgaatggagcgagc

SEQ ID NO: 441 - DNA, 89 bp, Artificial Sequence
  Description of Artificial Sequence: Synthetic oligonucleotide
ccattccctctttagccagagccggggtgtgcagacggcacttagggggcgctcggccaccacagggaagctgggtgaatggagcgagc

SEQ ID NO: 442 - DNA, 88 bp, Artificial Sequence
  Description of Artificial Sequence: Synthetic oligonucleotide
ccattccctctttagccagagccggggtgtgcagacggcactagggggcgctcggccaccacagggaagctgggtgaatggagcgagc

SEQ ID NO: 443 - DNA, 87 bp, Artificial Sequence
  Description of Artificial Sequence: Synthetic oligonucleotide
ccattccctctttagccagagccggggtgtgcagacggcagtcagggcgctcggccaccacagggaagctgggtgaatggagcgagc

SEQ ID NO: 444 - DNA, 87 bp, Artificial Sequence
  Description of Artificial Sequence: Synthetic oligonucleotide
ccattccctctttagccagagccggggtgtgcagacggcatagggggcgctcggccaccacagggaagctgggtgaatggagcgagc

SEQ ID NO: 445 - DNA, 84 bp, Artificial Sequence
  Description of Artificial Sequence: Synthetic oligonucleotide
ccattccctctttagccagagccggggtgtgcagacctagggggcgctcggccaccacagggaagctgggtgaatggagcgagc

SEQ ID NO: 446 - DNA, 83 bp, Artificial Sequence
  Description of Artificial Sequence: Synthetic oligonucleotide
ccattccctctttagccagagccggggtgtgcagacggcagggcgctcggccaccacagggaagctgggtgaatggagcgagc

SEQ ID NO: 447 - DNA, 83 bp, Artificial Sequence
  Description of Artificial Sequence: Synthetic oligonucleotide
ccattccctctttagccagagccggggtgtgcagactagggggcgctcggccaccacagggaagctgggtgaatggagcgagc

SEQ ID NO: 448 - DNA, 82 bp, Artificial Sequence
  Description of Artificial Sequence: Synthetic oligonucleotide
ccattccctctttagccagagccggggtgtgcagctagggggcgctcggccaccacagggaagctgggtgaatggagcgagc

SEQ ID NO: 449 - DNA, 81 bp, Artificial Sequence
  Description of Artificial Sequence: Synthetic oligonucleotide
ccattccctctttagccagagccggggtgtgcagaagggggcgctcggccaccacagggaagctgggtgaatggagcgagc

SEQ ID NO: 450 - DNA, 81 bp, Artificial Sequence
  Description of Artificial Sequence: Synthetic oligonucleotide
ccattccctctttagccagagccggggtgtgcactagggggcgctcggccaccacagggaagctgggtgaatggagcgagc

SEQ ID NO: 451 - DNA, 79 bp, Artificial Sequence
  Description of Artificial Sequence: Synthetic oligonucleotide
ccattccctctttagccagagccggggtgtgcagacggcagttcggccaccacagggaagctgggtgaatggagcgagc

SEQ ID NO: 452 - DNA, 78 bp, Artificial Sequence
  Description of Artificial Sequence: Synthetic oligonucleotide
ccattccctctttagccagagccggggtgtctagggggcgctcggccaccacagggaagctgggtgaatggagcgagc

SEQ ID NO: 453 - DNA, 77 bp, Artificial Sequence
  Description of Artificial Sequence: Synthetic oligonucleotide
ccattccctctttagccagagccggggtgtgcaggggcgctcggccaccacagggaagctgggtgaatggagcgagc

SEQ ID NO: 454 - DNA, 76 bp, Artificial Sequence
  Description of Artificial Sequence: Synthetic oligonucleotide
ccattccctctttagccagagccggggtgtgcagggcgctcggccaccacagggaagctgggtgaatggagcgagc

SEQ ID NO: 455 - DNA, 76 bp, Artificial Sequence
  Description of Artificial Sequence: Synthetic oligonucleotide
ccattccctctttagccagagccggggtgtgcagacggcagtcactacacagggaagctgggtgaatggagcgagc

SEQ ID NO: 456 - DNA, 76 bp, Artificial Sequence
  Description of Artificial Sequence: Synthetic oligonucleotide
ccattccctctttagccagagccggggtgtgcagacggctcggccaccacagggaagctgggtgaatggagcgagc

SEQ ID NO: 457 - DNA, 75 bp, Artificial Sequence
  Description of Artificial Sequence: Synthetic oligonucleotide
ccattccctctttagccagagccggggtgtgcagacgctcggccaccacagggaagctgggtgaatggagcgagc

SEQ ID NO: 458 - DNA, 73 bp, Artificial Sequence
  Description of Artificial Sequence: Synthetic oligonucleotide
ccattccctctttagccagagccggggtgggggcgctcggccaccacagggaagctgggtgaatggagcgagc

SEQ ID NO: 459 - DNA, 71 bp, Artificial Sequence
  Description of Artificial Sequence: Synthetic oligonucleotide
ccattccctctttagccagagccggggtgtgcgctcggccaccacagggaagctgggtgaatggagcgagc

SEQ ID NO: 460 - DNA, 71 bp, Artificial Sequence
  Description of Artificial Sequence: Synthetic oligonucleotide
ccattccctctttagccagagccggggtgtgcagacggcagtcacagggaagctgggtgaatggagcgagc

SEQ ID NO: 461 - DNA, 71 bp, Artificial Sequence
  Description of Artificial Sequence: Synthetic oligonucleotide
ccattccctctttagccagagccggggtgtgcagacggccaccacagggaagctgggtgaatggagcgagc

SEQ ID NO: 462 - DNA, 69 bp, Artificial Sequence
  Description of Artificial Sequence: Synthetic oligonucleotide
ccattccctctttagccagagccggggtgtgcagacggcagtcagggaagctgggtgaatggagcgagc

SEQ ID NO: 463 - DNA, 68 bp, Artificial Sequence
  Description of Artificial Sequence: Synthetic oligonucleotide
ccattccctctttagccagagccggggtgtgcaggccaccacagggaagctgggtgaatggagcgagc

SEQ ID NO: 464 - DNA, 68 bp, Artificial Sequence
  Description of Artificial Sequence: Synthetic oligonucleotide
ccattccctctttagccagagccggggtgtgcagaccaccacagggaagctgggtgaatggagcgagc

SEQ ID NO: 465 - DNA, 65 bp, Artificial Sequence
  Description of Artificial Sequence: Synthetic oligonucleotide
ccattccctctttagccagagccggggtgtgcagaccacagggaagctgggtgaatggagcgagc

SEQ ID NO: 466 - DNA, 58 bp, Artificial Sequence
  Description of Artificial Sequence: Synthetic oligonucleotide
ccattccctcttagtgactgctcggccaccacagggaagctgggtgaatggagcgagc